European Patent Application EP 4 600 256 A1, published August 13, 2025. Title: 呼吸道合胞病毒疫苗及其制备方法和应用. Applicant: 珠海丽凡达生物技术有限公司. Application CN. The sequence listing filed with the application follows.

SEQUENCE LISTING (103 sequences)

SEQ ID NO: 1 - protein, 227 aa, synthetic construct
DKTHTCPPCPAPELLGGPSVFLFPPKPKDTLMISRTPEVTCVVVDVSHEDPEVKFNWYVDGVEVHNAKTKPREEQYNSTYRVVSVLTVLHQDWLNGKEYKCKVSNKALPAPIEKTISKAKGQPREPQVYTLPPSREEMTKNQVSLTCLVKGFYPSDIAVEWESNGQPENNYKTTPPVLDSDGSFFLYSKLTVDKSRWQQGNVFSCSVMHEALHNHYTQKSLSLSPGK

SEQ ID NO: 2 - protein, 214 aa, synthetic construct
MEVSSVFIFPPKPKDVLTITLTPKVTCVVVDISKDDPEVQFSWFVDDVEVHTAQTQPREEQFNSTFRSVSELPIMHQDWLNGKEFKCRVNSAAFPAPIEKTISKTKGRPKAPQVYTIPPPKEQMAKDKVSLTCMITDFFPEDITVEWQWNGQPAENYKNTQPIMDTDGSYFVYSKLNVQKSNWEAGNTFTCSVLHEGLHNHHTEKSLSHSPGKE

SEQ ID NO: 3 - protein, 27 aa, synthetic construct
GYIPEAPRDGQAYVRKDGEWVLLSTFL

SEQ ID NO: 4 - protein, 28 aa, synthetic construct
GSGYIPRAPRDGQAYVRKDGEWVLLSTF

SEQ ID NO: 5 - protein, 81 aa, synthetic construct
GSYHADPSLVSFLTGLGCPNCIEYFTSQGLQSIYHLQNLTIEDLGALKIPEQYRMTIWRGLQDLKQGHDYSTAQQLLRSSS

SEQ ID NO: 6 - protein, 56 aa, synthetic construct
GSSGVRLWATRQAMLGQVHEVPEGWLIFVAEQEELYVRVQNGFRKVQLEARTPLPR

SEQ ID NO: 7 - protein, 31 aa, synthetic construct
SAIGGYIPEAPRDGQAYVRKDGEWVLLSTFL

SEQ ID NO: 8 - protein, 235 aa, synthetic construct
DEIMTSLKSVNGQIESLISPDGSRKNPARNCRDLKFCHPELKSGEYWVDPNQGCKLDAIKVFCNMETGETCISANPLNVPRKHWWTDSSAEKKHVWFGESMDGGFQFSYGNPELPEDVLDVQLAFLRLLSSRASQNITYHCKNSIAYMDQASGNVKKALKLMGSNEGEFKAEGNSKFTYTVLEDGCTKHTGEWSKTVFEYRTRKAVRLPIVDIAPYDIGGPDQEFGVDVGPVCFL

SEQ ID NO: 9 - protein, 244 aa, synthetic construct
ANVVRDRDLEVDTTLKSLSQQIENIRSPEGSRKNPARTCRDLKMCHSDWKSGEYWIDPNQGCNLDAIKVFCNMETGETCVYPTQPSVAQKNWYISKNPKDKRHVWFGESMTDGFQFEYGGQGSDPADVAIQLTFLRLMSTEASQNITYHCKNSVAYMDQQTGNLKKALLLKGSNEIEIRAEGNSRFTYSVTVDGCTSHTGAWGKTVIEYKTTKSSRLPIIDVAPLDVGAPDQEFGFDVGPVCFL

SEQ ID NO: 10 - protein, 245 aa, synthetic construct
SEPMDFKINTDEIMTSLKSVNGQIESLISPDGSRKNPARNCRDLKFCHPELKSGEYWVDPNQGCKLDAIKVFCNMETGETCISANPLNVPRKHWWTDSSAEKKHVWFGESMDGGFQFSYGNPELPEDVLDVQLAFLRLLSSRASQNITYHCKNSIAYMDQASGNVKKALKLMGSNEGEFKAEGNSKFTYTVLEDGCTKHTGEWSKTVFEYRTRKAVRLPIVDIAPYDIGGPDQEFGVDVGPVCFL

SEQ ID NO: 11 - protein, 64 aa, synthetic construct
NLQQFKNMIQCAGTRTWTAYINYGCYCGKGGSGTPVDKLDRCCYTHDHCYNQADSIPGCNPNIK

SEQ ID NO: 12 - protein, 32 aa, synthetic construct
MKQIEDKIEEILSKIYHIENEIARIKKLIGER

SEQ ID NO: 13 - RNA, 96 nt, synthetic construct
  source 1..96: mol_type = other RNA
atgaagcagatcgaggacaagatcgaggagatcttgtccaagatctaccacatagagaacgagatagctcggattaagaagctcattggcgagaga

SEQ ID NO: 14 - protein, 31 aa, synthetic construct
GEYFTLKIRGRKRFEMFRELNEALELKDAHA

SEQ ID NO: 15 - protein, 30 aa, synthetic construct
EEIFTLRIKGRSRYEMIKKLNDALELQESL

SEQ ID NO: 16 - RNA, 15 nt, synthetic construct
  source 1..15: mol_type = other RNA
gggagaaagcttacc

SEQ ID NO: 17 - RNA, 47 nt, synthetic construct
  source 1..47: mol_type = other RNA
gggaaataagagagaaaagaagagtaagaagaaatataagagccacc

SEQ ID NO: 18 - RNA, 57 nt, synthetic construct
  source 1..57: mol_type = other RNA
gggaaataagagagaaaagaagagtaagaagaaatataagaccccggcgccgccacc

SEQ ID NO: 19 - RNA, 74 nt, synthetic construct
  source 1..74: mol_type = other RNA
ggactagttataagactgactagcccgatgggcctcccaacgggccctcctcccctccttgcaccgagattaat

SEQ ID NO: 20 - RNA, 119 nt, synthetic construct
  source 1..119: mol_type = other RNA
tgataataggctggagcctcggtggccatgcttcttgccccttgggcctccccccagcccctcctccccttcctgcacccgtacccccgtggtctttgaataaagtctgagtgggcggc

SEQ ID NO: 21 - RNA, 119 nt, synthetic construct
  source 1..119: mol_type = other RNA
tgataataggctggagcctcggtggcctagcttcttgccccttgggcctccccccagcccctcctccccttcctgcacccgtacccccgtggtctttgaataaagtctgagtgggcggc

SEQ ID NO: 22 - protein, 499 aa, synthetic construct
MELLILKANAITTILTAVTFCFASGQNITEEFYQSTCSAVSKGYLSALRTGWYTSVITIELSNIKKNKCNGTDAKIKLIKQELDKYKNAVTELQLLMGGGSGGGSGGGSGSAIASGVAVCKVLHLEGEVNKIKSALLSTNKAVVSLSNGVSVLTFKVLDLKNYIDKQLLPILNKQSCSISNIETVIEFQQKNNRLLEITREFSVNAGVTTPVSTYMLTNSELLSLINDMPITNDQKKLMSNNVQIVRQQSYSIMCIIKEEVLAYVVQLPLYGVIDTPCWKLHTSPLCTTNTKEGSNICLTRTDRGWYCDNAGSVSFFPQAETCKVQSNRVFCDTMNSLTLPSEVNLCNVDIFNPKYDCKIMTSKTDVSSSVITSLGAIVSCYGKTKCTASNKNRGIIKTFSNGCDYVSNKGVDTVSVGNTLYYVNKQEGKSLYVKGEPIINFYDPLVFPSCEFCASISQVNEKINQSLSAIGGYIPEAPRDGQAYVRKDGEWVLLSTFL

SEQ ID NO: 23 - RNA, 1497 nt, synthetic construct
  source 1..1497: mol_type = other RNA
atggagcttctcatcctgaaggctaacgccattacgacaatactgaccgcggtcacgttctgctttgcgagcggacagaatatcactgaggagttctaccagtccacgtgcagcgccgtgtcaaagggctacctcagcgcgttgcggaccggctggtacacctccgttatcaccatcgagctgtccaacatcaagaagaacaagtgcaacgggacggacgccaagattaagcttatcaagcaggagcttgataagtataagaacgccgtcaccgagttgcagttgttgatggggggcggctccggtggtggtagcggaggtggcagcgggtccgcaatcgcgtctggggtagccgtttgcaaggtgctgcacttggagggagaagtcaacaagataaagtccgctctgctgagcacgaacaaggccgtggtcagtttgtcgaatggcgttagcgtcctgacgttcaaggtgctcgacctcaagaactatatcgacaagcagctgctgccgatactgaacaagcagagttgtagcatcagcaacatcgagaccgtgattgagttccagcagaagaacaatcgtctgctggaaatcactcgcgagttctcggtgaatgctggtgttacaactccggtcagcacctacatgctgaccaactcagagcttctgtcgttgattaacgacatgccgataaccaacgaccagaagaagctcatgagtaataatgttcagatcgtgcggcagcagtcgtatagtatcatgtgtatcataaaggaggaggtgttggcttacgtcgtacagctgccgctgtacggcgtgatcgacaccccctgctggaagctgcacacttccccgttgtgcactaccaacacgaaggaggggtcaaacatctgtttgacccgtaccgatcgtggttggtattgcgacaacgcgggaagtgtcagcttcttcccgcaggctgagacctgcaaggtccagtctaaccgggttttttgtgataccatgaactctctgacgttgccgtcagaggttaatctttgtaacgtcgatatcttcaatcccaagtacgattgtaagataatgacgtcaaagactgacgtgtcgtcatccgttataacgtctttaggtgccatcgtttcttgttacggcaagactaagtgtactgccagtaacaagaatcgaggcatcataaagacgtttagtaacggatgcgactacgtcagcaacaagggggtcgacaccgtgagcgtcgggaacacgttgtactacgtgaacaagcaggaggggaagtctctatacgtgaaaggcgagccgatcataaacttttatgatccgctcgtctttccgtcgtgtgagttttgtgcgagtatctcccaggtgaacgagaagattaaccagagtctctcggccatcgggggatacatccccgaagctccacgggacggccaggcctacgtccgtaaggacggagagtgggtcttgctgtccactttttta

SEQ ID NO: 24 - protein, 574 aa, synthetic construct
MELLILKANAITTILTAVTFCFASGQNITEEFYQSTCSAVSKGYLSALRTGWYTSVITIELSNIKKNKCNGTDAKIKLIKQELDKYKNAVTELQLLMQSTPATNNRARRELPRFMNYTLNNAKKTNVTLSKKRKRRFLGFLLGVGSAIASGVAVSKVLHLEGEVNKIKSALLSTNKAVVSLSNGVSVLTSKVLDLKNYIDKQLLPIVNKQSCSISNIETVIEFQQKNNRLLEITREFSVNAGVTTPVSTYMLTNSELLSLINDMPITNDQKKLMSNNVQIVRQQSYSIMSIIKEEVLAYVVQLPLYGVIDTPCWKLHTSPLCTTNTKEGSNICLTRTDRGWYCDNAGSVSFFPQAETCKVQSNRVFCDTMNSLTLPSEVNLCNVDIFNPKYDCKIMTSKTDVSSSVITSLGAIVSCYGKTKCTASNKNRGIIKTFSNGCDYVSNKGVDTVSVGNTLYYVNKQEGKSLYVKGEPIINFYDPLVFPSDEFDASISQVNEKINQSLAFIRKSDELLHNVNAVKSTTNIMITTIIIVIIVILLSLIAVGLLLYCKARSTPVTLSKDQLSGINNIAFSN

SEQ ID NO: 25 - RNA, 1725 nt, synthetic construct
  source 1..1725: mol_type = other RNA
atggaactgctgatcctgaaggccaacgccatcaccaccatcctgacagccgttacattctgcttcgccagcggacagaacatcaccgaggaattctaccagagcacctgcagcgccgtgagcaagggctacctgagcgccctgagaactggatggtacacaagcgtgattaccatcgagctgtctaatatcaagaagaacaagtgtaatggcaccgacgccaaaatcaaactgatcaagcaggagcttgataagtacaagaacgctgtgacagagctgcaactgctgatgcagagcacccctgctacaaacaacagagccaggcgggaactgcctagattcatgaactacaccctgaacaatgctaaaaagaccaatgtgacactgagcaagaagcggaaaagacggttcctgggatttctgctgggcgtcggcagcgctatcgcctccggcgtggccgtgagcaaggtgctgcacctggaaggagaagtgaacaagatcaaatctgcactgctgagcacaaataaggccgtggtgagcctgagcaacggcgtgtccgtgctgacctccaaggtgctggacctgaagaattacatcgacaaacagctgctgcctatcgtgaacaagcagagctgcagcatcagcaacatcgagacagtgattgaatttcagcagaagaacaaccggctgcttgagatcactcgggaattcagcgtgaacgccggcgtcacaacccctgtgtctacctacatgctgaccaatagcgagctgctgagcctgattaacgacatgcctatcaccaacgaccagaaaaagctgatgagcaacaacgtgcaaatcgtgcgccagcagagctacagcatcatgagcatcatcaaagaggaagtgctggcttacgtggtccaactgccactgtacggcgttattgacacaccatgttggaagctgcacaccagccctctgtgcaccaccaacaccaaggaaggcagcaacatctgcctgaccagaaccgatagaggctggtattgtgacaacgctggatccgtgtccttcttccctcaggccgagacatgtaaagtgcagagtaatagagtgttttgcgacaccatgaacagcctgacactgccttctgaggtgaatctgtgcaacgtggacatcttcaaccccaagtacgattgcaagatcatgacctctaagacagatgtgagcagctctgtgatcacaagcctgggcgccatcgtgagctgttacggcaagaccaagtgcaccgccagcaataaaaaccggggcatcatcaaaacctttagcaacggctgcgactacgtctctaacaagggcgtggataccgtgagcgtggggaacaccctatactacgtgaacaaacaggagggcaagtccctgtacgtgaagggagagcccatcatcaacttctacgaccccctggtgttccccagcgacgagttcgacgcctctatcagccaggtgaacgagaagatcaaccagtccctcgccttcatccggaagagcgacgagctgctccacaacgtcaatgccgtgaagagcaccaccaacatcatgatcacaacgatcatcatcgtgatcatcgtgattctgctgtcccttatcgccgtaggcctgctgctgtactgcaaggccagaagcacacctgttaccctgagcaaggaccagctgtctggcatcaacaatatcgctttcagcaattga

SEQ ID NO: 26 - protein, 544 aa, synthetic construct
MELLILKANAITTILTAVTFCFASGQNITEEFYQSTCSAVSKGYLSALRTGWYTSVITIELSNIKKNKCNGTDAKIKLIKQELDKYKNAVTELQLLMQSTPATNNRARRELPRFMNYTLNNAKKTNVTLSKKRKRRFLGFLLGVGSAIASGVAVCKVLHLEGEVNKIKSALLSTNKAVVSLSNGVSVLTFKVLDLKNYIDKQLLPILNKQSCSISNIETVIEFQQKNNRLLEITREFSVNAGVTTPVSTYMLTNSELLSLINDMPITNDQKKLMSNNVQIVRQQSYSIMCIIKEEVLAYVVQLPLYGVIDTPCWKLHTSPLCTTNTKEGSNICLTRTDRGWYCDNAGSVSFFPQAETCKVQSNRVFCDTMNSLTLPSEVNLCNVDIFNPKYDCKIMTSKTDVSSSVITSLGAIVSCYGKTKCTASNKNRGIIKTFSNGCDYVSNKGVDTVSVGNTLYYVNKQEGKSLYVKGEPIINFYDPLVFPSDEFDASISQVNEKINQSLAFIRKSDELLSAIGGYIPEAPRDGQAYVRKDGEWVLLSTFL

SEQ ID NO: 27 - RNA, 1635 nt, synthetic construct
  source 1..1635: mol_type = other RNA
atggaactgctcattctgaaagccaacgccatcaccaccatcctgaccgccgtcacattttgcttcgccagcggccagaacatcacagaggagttctaccagagcacctgtagcgccgtgtccaagggctacctgagcgccctgcggaccggctggtatacaagcgtgatcaccatcgagctgagcaacatcaaaaaaaacaagtgtaacggtacagatgctaaaatcaagctgatcaagcaggagctcgacaagtacaagaacgcagttaccgagctccagctgctgatgcagagcacccctgctacaaacaaccgcgccagaagggaactgcctagattcatgaactacaccctgaacaacgccaagaagacaaatgtgaccctgagcaagaaaagaaagcggagattcctgggcttcctgctgggcgtgggcagcgccatcgccagcggggtcgccgtctgcaaagtgctgcacctggaaggcgaagtgaacaagattaaatctgctctgctgagcaccaacaaggctgttgtgtccctgagcaatggagtttctgtgctgacctttaaggtgctggatctgaagaattacatcgacaagcagctgctgcctatcctgaacaagcagagttgcagcattagcaatatcgagaccgtgatcgagtttcagcagaaaaataacagactgctggaaatcacaagagagttcagcgtgaacgctggcgtgacaacccctgtgtctacctacatgctgacaaacagcgagctgctgagcctgatcaacgacatgcctattaccaatgaccagaagaaactgatgagcaacaacgtgcaaatcgtgcggcagcagtcctacagcatcatgtgcatcatcaaggaggaagtgctggcttatgtggtgcagctgcccctgtatggcgtcatcgacaccccatgctggaagctgcacacgagccctctgtgtacaacaaacacaaaggaaggcagcaacatctgcctgacccggaccgatagaggctggtactgtgataacgccggctctgtgagcttcttcccacaggccgaaacctgcaaggtgcagagcaacagagtgttctgcgacaccatgaacagcctgaccctgcctagcgaggtgaatctgtgcaacgtggacatcttcaaccccaagtacgactgcaagatcatgacctccaaaaccgacgtgtctagcagcgtgatcaccagcctgggagccatcgtgtcctgctacggcaagaccaagtgcacagcctctaacaagaatcggggcatcatcaagacctttagcaatggctgtgactacgtgtctaataagggcgtcgatactgtgagtgtcggcaacaccctgtactacgtgaacaagcaagagggaaagtccctgtacgtgaagggcgagcctatcatcaacttctacgaccccctggtgttccccagcgacgagttcgacgcctctatctcccaggtgaacgagaagatcaaccagagcctggccttcatcagaaagtctgatgagctgctctcagccattggaggatacatccccgaggcccctagagatggccaagcctacgtgcggaaggacggcgaatgggtgctgctgtctacattcctgtga

SEQ ID NO: 28 - protein, 526 aa, synthetic construct
MELLILKANAITTILTAVTFCFASGQNITEEFYQSTCSAVSKGYLSALRTGWYTSVITIELSNIKKNKCNGTDAKIKLIKQELDKYKNAVTELQLLMGGGSGGGSGGGSGSAIASGVAVCKVLHLEGEVNKIKSALLSTNKAVVSLSNGVSVLTFKVLDLKNYIDKQLLPILNKQSCSISNIETVIEFQQKNNRLLEITREFSVNAGVTTPVSTYMLTNSELLSLINDMPITNDQKKLMSNNVQIVRQQSYSIMCIIKEEVLAYVVQLPLYGVIDTPCWKLHTSPLCTTNTKEGSNICLTRTDRGWYCDNAGSVSFFPQAETCKVQSNRVFCDTMNSLTLPSEVNLCNVDIFNPKYDCKIMTSKTDVSSSVITSLGAIVSCYGKTKCTASNKNRGIIKTFSNGCDYVSNKGVDTVSVGNTLYYVNKQEGKSLYVKGEPIINFYDPLVFPSCEFCASISQVNEKINQSLAFIRKSDELLHNVNAVKSTTNIMITTMKQIEDKIEEILSKIYHIENEIARIKKLIGER

SEQ ID NO: 29 - RNA, 1581 nt, synthetic construct
  source 1..1581: mol_type = other RNA
atggaactgctgatcctgaaagccaacgccatcaccaccatcctcaccgccgttaccttctgcttcgcctctggccagaacatcaccgaagagttctaccaaagcacctgcagcgccgtgtccaagggctacctgtctgctctgagaacaggctggtacacaagcgtgatcacaatcgagctgtctaacatcaagaagaacaaatgcaacggcaccgacgccaagattaagctgattaagcaggagctggacaagtacaagaatgccgtgacagagctgcagctgcttatgggcggaggcagcggcggcggctccggtggcggcagcggatctgccatcgcctccggcgtcgccgtgtgcaaggtgctgcacctggaaggcgaggtgaacaagatcaagagcgctctgctcagcacaaacaaggccgtggtgtctctgtccaacggcgtttccgtgctgacctttaaggtgctggacctgaagaattacatcgacaagcagctgctgcctatcctgaacaagcaaagctgtagcatcagcaatattgagacagtgatcgagtttcagcagaagaacaaccggctgctggaaatcacacgggaatttagcgtgaatgccggcgtgaccacacctgtgtctacatacatgctgaccaatagcgagctgctgtctttgatcaacgacatgcctatcacaaatgatcagaaaaagctgatgagcaacaacgtgcaaatcgtgaggcagcagtcatatagcatcatgtgcatcatcaaagaggaagtgctggcctacgtcgtgcagctgccactgtacggcgtcatcgacacaccctgctggaagctgcacacctcccctctgtgcacaaccaacaccaaggaagggtccaacatctgcctgaccagaaccgatagaggctggtactgcgacaatgctggctcagtgagcttcttcccccaggctgaaacctgtaaagtgcagagcaacagagtgttctgcgacaccatgaacagcctgacactgcctagcgaggtgaacctgtgcaatgtggacatcttcaaccccaagtatgattgtaaaatcatgaccagcaagaccgacgtgtccagcagcgtgatcaccagcctgggagccatcgtgagctgctacggcaaaacaaagtgcaccgcctctaacaagaacagaggaattatcaaaaccttcagcaacggctgtgactacgttagcaacaagggagtggatacagtgagcgtgggaaataccctgtactacgtgaacaaacaggaaggcaagtccctgtacgtgaagggcgaacccattatcaacttctacgaccctctggtgttcccaagctgcgagttttgtgccagcatctctcaggtgaacgagaagatcaaccagagcctggccttcatcagaaagagtgatgagctgctgcacaacgtgaacgccgtgaagagcaccacgaatatcatgatcaccaccatgaagcagatcgaggacaagatcgaggagatcttgtccaagatctaccacatagagaacgagatagctcggattaagaagctcattggcgagagatga

SEQ ID NO: 30 - protein, 535 aa, synthetic construct
MELLILKANAITTILTAVTFCFASGQNITEEFYQSTCSAVSKGYLSALRTGWYTSVITIELSNIKENKCNGTDAKVKLIKQELDKYKNAVTELQLLMQSTPATGSGSAICSGVAVCKVLHLEGEVNKIKSALLSTNKAVVSLSNGVSVLTFKVLDLKNYIDKQLLPILNKQSCSISNIETVIEFQQKNNRLLEITREFSVNAGVTTPVSTYMLTNSELLSLINDMPITNDQKKLMSNNVQIVRQQSYSIMCIIKEEVLAYVVQLPLYGVIDTPCWKLHTSPLCTTNTKEGSNICLTRTDRGWYCDNAGSVSFFPQAETCKVQSNRVFCDTMNSRTLPSEVNLCNVDIFNPKYDCKIMTSKTDVSSSVITSLGAIVSCYGKTKCTASNKNRGIIKTFSNGCDYVSNKGVDTVSVGNTLYCVNKQEGKSLYVKGEPIINFYDPLVFPSDEFDASISQVNEKINQSLAFIRKSDELLHNVNAGKSTTNIMITTIIIVIIVILLSLIAVGLLLYCKARSTPVTLSKDQLSGINNIAFSN

SEQ ID NO: 31 - RNA, 1608 nt, synthetic construct
  source 1..1608: mol_type = other RNA
atggaactgctcattttgaaggcaaacgctatcacgacaatactcactgcagtgaccttctgttttgcctcaggccagaacataaccgaggagttttatcaatctacatgcagcgctgtatctaaaggctacctgagtgcgctccgcacaggatggtacacctccgtgatcaccatcgagctcagcaatattaaagagaacaagtgcaatggtaccgacgctaaagtcaaacttatcaagcaggaactcgacaaatataagaacgctgtgaccgagctgcagttattgatgcagagtacacctgccaccgggtcgggctctgccatttgctccggcgtggctgtatgtaaagttctccacctcgagggagaggttaataagattaagtcggccctgctgagtactaacaaagcagtggtgtcgctgagtaacggagtaagtgtgttaacatttaaggtgctggacctcaagaattatattgacaaacagttgcttcctattctaaacaaacagagctgttcaataagtaatattgaaactgttattgagtttcagcagaagaacaacaggcttcttgagattacacgcgagttcagtgtcaatgccggcgttacaacacccgtgtctacctacatgctgacgaattctgagcttctctctctcataaacgacatgcccattacgaatgaccaaaagaaacttatgtccaacaacgtgcagattgtgcgacagcaatcctatagcattatgtgtatcatcaaggaagaggtactcgcttatgttgtgcagctaccactctatggtgtgattgacaccccctgttggaagctgcataccagtccactctgcaccactaacacaaaggaagggagcaatatttgcctcactcgaaccgacagggggtggtattgcgataatgcgggctccgtgtccttctttccacaggctgaaacttgtaaggtacagtcaaaccgcgtgttctgtgatactatgaattctcgtactcttcccagcgaggttaatctctgcaacgtcgacattttcaatcctaaatatgactgcaagatcatgaccagcaagaccgacgtctccagctcagtaatcactagcctaggggccattgtaagctgctatggcaaaaccaagtgtactgcctctaataagaacagaggcataattaaaaccttttcaaatggctgtgactatgtgtcgaataagggcgtcgacacggtctcagtagggaataccctctactgcgttaacaaacaggaaggcaaatccctttatgtaaagggcgagcccatcataaatttctacgacccacttgtgttccccagtgatgaattcgatgcatcaatctcccaggtgaacgaaaagatcaatcaatcccttgcttttatacgaaagtcagatgaactcctgcataacgtgaatgctgggaaatctacaaccaacatcatgatcactaccatcattattgtgattatcgtaattctgctatccttgattgctgtcgggctgcttctgtactgtaaggccagatcgacgcctgtgaccctttcaaaagaccaacttagcggtatcaataatattgcctttagcaattga

SEQ ID NO: 32 - protein, 544 aa, synthetic construct; identical to SEQ ID NO: 26

SEQ ID NO: 33 - RNA, 1635 nt, synthetic construct; identical to SEQ ID NO: 27
  source 1..1635: mol_type = other RNA

SEQ ID NO: 34 - protein, 530 aa, synthetic construct
MELLILKANAITTILTAVTFCFASGQNITEEFYQSTCSAVSKGYLGALRTGWYTSVITIELSNIKKIKCNGTDAKIKLIKQELDKYKNAVTDLQLLMQSTPATNNRARRGSFLGFLLGVGSAICSGVAVCKVLHLEGEVNKIKSALLSTNKAVVSLSNGVSVLTFKVLDLKNYIDKQLLPILNKQSCSIPNIETVIEFQQKNNRLLEITREFSVNAGVTTPVSTYMLTNSELLSLINDMPITNDQKKLMSNNVQIVRQQSYSIMCIIKEEVLAYVVQLPLYGVIDTPCWKLHTSPLCTTNTKEGSNICLTRTDRGWYCDNAGSVSFFPQAETCKVQSNRVFCDTMNSLTLPSEVNLCNVDIFNPKYDCKIMTSKTDVSSSVITSLGAIVSCYGKTKCTASNKNRGIIKTFSNGCDYVSNKGVDTVSVGNTLYCVNKQEGQSLYVKGEPIINFYDPLVFPSDEFDASISQVNEKINQSLAFIRKSDELLHNVNAVKSTTNSAIGGYIPEAPRDGQAYVRKDGEWVLLSTFL

SEQ ID NO: 35 - RNA, 1497 nt, synthetic construct
  source 1..1497: mol_type = other RNA
atggaactgctgatcctgaaggccaacgccatcaccaccatcctgacagccgttacattctgcttcgccagcggacagaacatcaccgaggaattctaccagagcacctgcagcgccgtgagcaagggctacctgggcgccctgagaactggatggtacacaagcgtgattaccatcgagctgtctaatatcaagaagatcaagtgtaatggcaccgacgccaaaatcaaactgatcaagcaggagcttgataagtacaagaacgctgtgacagatctgcaactgctgatgcagagcacccctgctacaggctctggcagcgctatctgctccggcgtggccgtgtgcaaggtgctgcacctggaaggagaagtgaacaagatcaaatctgcactgctgagcacaaataaggccgtggtgagcctgagcaacggcgtgtccgtgctgaccttcaaggtgctggacctgaagaattacatcgacaaacagctgctgcctatcctgaacaagcagagctgcagcatccccaacatcgagacagtgattgaatttcagcagaagaacaaccggctgcttgagatcactcgggaattcagcgtgaacgccggcgtcacaacccctgtgtctacctacatgctgaccaatagcgagctgctgagcctgattaacgacatgcctatcaccaacgaccagaaaaagctgatgagcaacaacgtgcaaatcgtgcgccagcagagctacagcatcatgtgcatcatcaaagaggaagtgctggcttacgtggtccaactgccactgtacggcgttattgacacaccatgttggaagctgcacaccagccctctgtgcaccaccaacaccaaggaaggcagcaacatctgcctgaccagaaccgatagaggctggtattgtgacaacgctggatccgtgtccttcttccctcaggccgagacatgtaaagtgcagagtaatagagtgttttgcgacaccatgaacagcctgacactgccttctgaggtgaatctgtgcaacgtggacatcttcaaccccaagtacgattgcaagatcatgacctctaagacagatgtgagcagctctgtgatcacaagcctgggcgccatcgtgagctgttacggcaagaccaagtgcaccgccagcaataaaaaccggggcatcatcaaaacctttagcaacggctgcgactacgtctctaacaagggcgtggataccgtgagcgtggggaacaccctatactgcgtgaacaaacaggagggccagtccctgtacgtgaagggagagcccatcatcaacttctacgaccccctggtgttccccagctgcgagttctgcgcctctatcagccaggtgaacgagaagatcaaccagtccctcgccttcatctctgccatcggcggctatatccctgaggcccctagagatggccaggcctacgtcagaaaggacggcgaatgggtgctgctgtctacattcctgtga

SEQ ID NO: 36 - RNA, 684 nt, synthetic construct
  source 1..684: mol_type = other RNA
gataagacacatacctgtcccccatgccccgccccagagctgctgggaggcccctctgtgttcctgttccccccaaagccaaaggataccctgatgatcagtcggaccccagaggtgacctgcgtggtggtggacgtgagccacgaggaccccgaggtgaaattcaattggtacgtggatggggtcgaggtgcacaacgccaagaccaaaccacgggaagagcagtacaactccacatacagagtggtgtccgtgctgacagtgctgcaccaggactggctgaatggcaaggagtataaatgcaaggtgagcaacaaggccctgcccgccccaatcgaaaaaactatttccaaggccaagggacagcccagagagccccaggtctacacactgcctccaagtagagaagagatgaccaagaaccaggtgtccctgacctgtctggtcaagggcttctacccatccgatatcgccgtggaatgggagtccaacggccagcctgagaacaactacaagaccacccctccagtgctggattctgacggctccttcttcctgtacagcaagctgaccgtggacaagtcccgctggcagcaggggaatgtgttctcttgtagcgtgatgcacgaggccctgcacaaccactacactcagaagagcctgtctctgtcccccgggaaataa

SEQ ID NO: 37 - RNA, 84 nt, synthetic construct
  source 1..84: mol_type = other RNA
ggctatatccctgaggcccctagagacggccaggcctacgtgaggaaggacggagagtgggtgctgctgtccacttttctgtga

SEQ ID NO: 38 - RNA, 246 nt, synthetic construct
  source 1..246: mol_type = other RNA
ggctcctaccacgccgaccctagcctggtgtcattcctgaccggcctggggtgccctaactgtatcgagtacttcaccagccagggcctgcagagcatctaccacctgcagaacctgaccatcgaggacctgggcgccctgaagattcctgagcagtatagaatgacaatctggcggggcctgcaggacctgaagcagggccacgattacagtacagcacagcagctgctgaggtcctcatcctga

SEQ ID NO: 39 - RNA, 708 nt, synthetic construct
  source 1..708: mol_type = other RNA
gatgagatcatgacctctctgaagtctgtgaacgggcagatcgagagcctgatctctcccgatggaagcagaaagaatcccgcccgcaactgccgtgacctgaagttctgccacccagagctgaagtctggggagtactgggtggatcctaatcagggctgcaagctggacgctatcaaggtgttttgtaacatggagaccggcgagacctgtatttccgccaaccctctgaatgtcccaaggaagcactggtggacagacagctcagccgagaagaagcatgtgtggttcggggaatccatggacgggggcttccagtttagctatggaaatcccgagctgccagaggacgtgctggacgtgcagctggccttcctgcggctgctgagctctcgcgccagccagaatattacctaccactgtaagaattccatcgcctacatggaccaggccagcggcaacgtcaagaaggcactgaagctgatgggcagcaacgaaggggaattcaaagccgaggggaactccaaatttacctacaccgtgctggaagacggctgcaccaagcacaccggggagtggtccaagaccgtgtttgagtacagaacacgcaaggccgtgaggctgcctatcgtggatatcgccccctacgacattggggggcctgaccaggagttcggcgtggatgtggggcccgtgtgcttcctgtga

SEQ ID NO: 40 - RNA, 194 nt, synthetic construct
  source 1..194: mol_type = other RNA
aacctgcagcagttcaaaaacatgatccagtgcgccggcaccagaacctggaccgcctacatcaattacggctgctactgtggcaaaggcggcagcggcacacccgtggataagctggataggtgctgttacacacacgatcactgctacaaccaggccgacagcatccctggctgcaaccctaacatcaagtg

SEQ ID NO: 41 - RNA, 96 nt, synthetic construct
  source 1..96: mol_type = other RNA
ggcgagtactttaccctgaagatccggggcaggaagcggttcgagatgtttagggagctgaatgaggccctggagctgaaggacgcccacgcctga

SEQ ID NO: 42 - RNA, 645 nt, synthetic construct
  source 1..645: mol_type = other RNA
atggaagtgagcagcgtgtttatcttcccaccaaagcccaaggatgtgctgaccatcaccctgacccccaaggtgacctgtgtggtggtggatatcagcaaggacgaccccgaggtgcagttctcttggtttgtggacgatgtggaggtgcacaccgcccagactcagcccagggaggagcagttcaattccacattccggagcgtgtctgagctgcccatcatgcaccaggactggctgaacgggaaggagtttaaatgcagggtgaactctgccgccttccccgcccccatcgagaagaccatttccaagaccaagggcaggcccaaggctccccaggtgtacaccattccccctcctaaggagcagatggccaaggacaaggtctccctgacttgtatgatcaccgatttctttcccgaggacattaccgtggaatggcagtggaacggccagcctgccgagaattataagaacacacagccaatcatggacacagacggctcttacttcgtgtatagtaagctgaatgtgcagaagtccaattgggaagccgggaacactttcacatgtagcgtcctgcacgagggcctgcacaatcaccacacagagaagagcctgagtcactcccccggcaaggaatga

SEQ ID NO: 43 - RNA, 90 nt, synthetic construct
  source 1..90: mol_type = other RNA
ggaagcggctacatcccaagagccccaagagatggccaggcctatgtgagaaaggatggcgaatgggtgctgctgagcactttcctgtga

SEQ ID NO: 44 - RNA, 171 nt, synthetic construct
  source 1..171: mol_type = other RNA
ggatcctccggcgtgagactgtgggccacccggcaggccatgctggggcaggtgcacgaggtgccagagggctggctgatttttgtggctgaacaggaggaactgtacgtgagagtgcagaatggatttagaaaggtgcagctggaggccaggacacccctgccaagataa

SEQ ID NO: 45 - RNA, 546 nt, synthetic construct
  source 1..546: mol_type = other RNA
ggcggctccaacaccaactggaaaaccctgtatgaggtcaagagcgaaaacctggggcagggggataagcctgactacttcagcagcgtggctaccgtggtgtacctgaggaaagagaactgcatgtaccaggcctgccccacccaggactgtaacaagaaggtgatcgaccagcagaacggcctgtatcgatgcgaaaagtgcgatactgaattccccaacttcaagtatcgcatgatcctgtccgtgaacatcgccgacttccaggagaaccagtgggtgacctgcttccaggagtccgccgaggccatcctggggcagaacgccgcctacctgggcgagctgaaagacaagaatgaacaggccttcgaggaggtgttccagaacgctaattttcgcagcttcatcttcagagtgcgggtgaaggtggagacatataacgacgagagcagaattaaggctacagtgatggacgtgaagcctgtggactaccgcgaatacgggagacggctggtgatgtctatccgacgcagcgccctgatgtga

SEQ ID NO: 46 - RNA, 90 nt, synthetic construct
  source 1..90: mol_type = other RNA
ggcgagatcgccgccatcaagcaggagatcgccgccatcaagaaggagatcgccgccatcaagtgggaaattgccgccatcaagcagtga

SEQ ID NO: 47 - RNA, 93 nt, synthetic construct
  source 1..93: mol_type = other RNA
gaggagattttcacactgaggatcaagggccggtccagatacgagatgatcaagaagctgaatgacgccctggagctgcaggagagcctgtga

SEQ ID NO: 48 - protein, 16 aa, synthetic construct
GGGGSLVPRGSGGGGS

SEQ ID NO: 49 - protein, 6 aa, synthetic construct
GSGSGS

SEQ ID NO: 50 - protein, 15 aa, synthetic construct
GGGGSLVPRGSGGGG

SEQ ID NO: 51 - protein, 11 aa, synthetic construct
GGSGGHMGSGG

SEQ ID NO: 52 - protein, 11 aa, synthetic construct
GGSGGSGGSGG

SEQ ID NO: 53 - protein, 14 aa, synthetic construct
GSGGGGSGGGGSGS

SEQ ID NO: 54 - protein, 8 aa, synthetic construct
GSGSGSGS

SEQ ID NO: 55 - protein, 18 aa, synthetic construct
GGGSEGGGSEGGGSEGGG

SEQ ID NO: 56 - protein, 8 aa, synthetic construct
AAGAATAA

SEQ ID NO: 57 - protein, 5 aa, synthetic construct
GGSSG

SEQ ID NO: 58 - protein, 11 aa, synthetic construct
GSGGGTGGGSG

SEQ ID NO: 59 - protein, 12 aa, synthetic construct
GSGSGSGSGGSG

SEQ ID NO: 60 - protein, 14 aa, synthetic construct
GSGGSGSGGSGGSG

SEQ ID NO: 61 - protein, 14 aa, synthetic construct
GSGGSGGSGGSGGS

SEQ ID NO: 62 - protein, 546 aa, synthetic construct
MELLILKANAITTILTAVTFCFASGQNITEEFYQSTCSAVSKGYLSALRTGWYTSVITIELSNIKKNKCNGTDAKIKLIKQELDKYKNAVTELQLLMGGGSGGGSGGGSGSAIASGVAVCKVLHLEGEVNKIKSALLSTNKAVVSLSNGVSVLTFKVLDLKNYIDKQLLPILNKQSCSISNIETVIEFQQKNNRLLEITREFSVNAGVTTPVSTYMLTNSELLSLINDMPITNDQKKLMSNNVQIVRQQSYSIMCIIKEEVLAYVVQLPLYGVIDTPCWKLHTSPLCTTNTKEGSNICLTRTDRGWYCDNAGSVSFFPQAETCKVQSNRVFCDTMNSLTLPSEVNLCNVDIFNPKYDCKIMTSKTDVSSSVITSLGAIVSCYGKTKCTASNKNRGIIKTFSNGCDYVSNKGVDTVSVGNTLYYVNKQEGKSLYVKGEPIINFYDPLVFPSCEFCASISQVNEKINQSLAFIRKSDELLHNVNAVKSTTNIMITTIIIVIIVILLSLIAVGLLLYCSAIGGYIPEAPRDGQAYVRKDGEWVLLSTFL

SEQ ID NO: 63 - RNA, 1641 nt, synthetic construct
  source 1..1641: mol_type = other RNA
atggaactgctgatcctgaaagccaacgccatcaccaccatcctcaccgccgttaccttctgcttcgcctctggccagaacatcaccgaagagttctaccaaagcacctgcagcgccgtgtccaagggctacctgtctgctctgagaacaggctggtacacaagcgtgatcacaatcgagctgtctaacatcaagaagaacaaatgcaacggcaccgacgccaagattaagctgattaagcaggagctggacaagtacaagaatgccgtgacagagctgcagctgcttatgggcggaggcagcggcggcggctccggtggcggcagcggatctgccatcgcctccggcgtcgccgtgtgcaaggtgctgcacctggaaggcgaggtgaacaagatcaagagcgctctgctcagcacaaacaaggccgtggtgtctctgtccaacggcgtttccgtgctgacctttaaggtgctggacctgaagaattacatcgacaagcagctgctgcctatcctgaacaagcaaagctgtagcatcagcaatattgagacagtgatcgagtttcagcagaagaacaaccggctgctggaaatcacacgggaatttagcgtgaatgccggcgtgaccacacctgtgtctacatacatgctgaccaatagcgagctgctgtctttgatcaacgacatgcctatcacaaatgatcagaaaaagctgatgagcaacaacgtgcaaatcgtgaggcagcagtcatatagcatcatgtgcatcatcaaagaggaagtgctggcctacgtcgtgcagctgccactgtacggcgtcatcgacacaccctgctggaagctgcacacctcccctctgtgcacaaccaacaccaaggaagggtccaacatctgcctgaccagaaccgatagaggctggtactgcgacaatgctggctcagtgagcttcttcccccaggctgaaacctgtaaagtgcagagcaacagagtgttctgcgacaccatgaacagcctgacactgcctagcgaggtgaacctgtgcaatgtggacatcttcaaccccaagtatgattgtaaaatcatgaccagcaagaccgacgtgtccagcagcgtgatcaccagcctgggagccatcgtgagctgctacggcaaaacaaagtgcaccgcctctaacaagaacagaggaattatcaaaaccttcagcaacggctgtgactacgttagcaacaagggagtggatacagtgagcgtgggaaataccctgtactacgtgaacaaacaggaaggcaagtccctgtacgtgaagggcgaacccattatcaacttctacgaccctctggtgttcccaagctgcgagttttgtgccagcatctctcaggtgaacgagaagatcaaccagagcctggccttcatcagaaagagtgatgagctgctgcacaacgtgaacgccgtgaagagcaccacgaatatcatgatcaccaccatcatcatcgtgatcatcgtgatcctgctgagcttaatcgcagttggcctgctcctgtattgttccgctattggcggatacatccctgaggcccctagagatggccaggcctacgtgcggaaggacggcgagtgggtcctgttgtctaccttcctgtga

SEQ ID NO: 64 - protein, 515 aa, synthetic construct
MELLILKANAITTILTAVTFCFASGQNITEEFYQSTCSAVSKGYLSALRTGWYTSVITIELSNIKKNKCNGTDAKIKLIKQELDKYKNAVTELQLLMGGGSGGGSGGGSGSAIASGVAVCKVLHLEGEVNKIKSALLSTNKAVVSLSNGVSVLTFKVLDLKNYIDKQLLPILNKQSCSISNIETVIEFQQKNNRLLEITREFSVNAGVTTPVSTYMLTNSELLSLINDMPITNDQKKLMSNNVQIVRQQSYSIMCIIKEEVLAYVVQLPLYGVIDTPCWKLHTSPLCTTNTKEGSNICLTRTDRGWYCDNAGSVSFFPQAETCKVQSNRVFCDTMNSLTLPSEVNLCNVDIFNPKYDCKIMTSKTDVSSSVITSLGAIVSCYGKTKCTASNKNRGIIKTFSNGCDYVSNKGVDTVSVGNTLYYVNKQEGKSLYVKGEPIINFYDPLVFPSCEFCASISQVNEKINQSLAFIRKSDELLHNVNAVKSTTNIMITTIIIVIIVILLSLIAVGLLLYC

SEQ ID NO: 65 - RNA, 1548 nt, synthetic construct
  source 1..1548: mol_type = other RNA
atggaactgctgatcctgaaagccaacgccatcaccaccatcctcaccgccgttaccttctgcttcgcctctggccagaacatcaccgaagagttctaccaaagcacctgcagcgccgtgtccaagggctacctgtctgctctgagaacaggctggtacacaagcgtgatcacaatcgagctgtctaacatcaagaagaacaaatgcaacggcaccgacgccaagattaagctgattaagcaggagctggacaagtacaagaatgccgtgacagagctgcagctgcttatgggcggaggcagcggcggcggctccggtggcggcagcggatctgccatcgcctccggcgtcgccgtgtgcaaggtgctgcacctggaaggcgaggtgaacaagatcaagagcgctctgctcagcacaaacaaggccgtggtgtctctgtccaacggcgtttccgtgctgacctttaaggtgctggacctgaagaattacatcgacaagcagctgctgcctatcctgaacaagcaaagctgtagcatcagcaatattgagacagtgatcgagtttcagcagaagaacaaccggctgctggaaatcacacgggaatttagcgtgaatgccggcgtgaccacacctgtgtctacatacatgctgaccaatagcgagctgctgtctttgatcaacgacatgcctatcacaaatgatcagaaaaagctgatgagcaacaacgtgcaaatcgtgaggcagcagtcatatagcatcatgtgcatcatcaaagaggaagtgctggcctacgtcgtgcagctgccactgtacggcgtcatcgacacaccctgctggaagctgcacacctcccctctgtgcacaaccaacaccaaggaagggtccaacatctgcctgaccagaaccgatagaggctggtactgcgacaatgctggctcagtgagcttcttcccccaggctgaaacctgtaaagtgcagagcaacagagtgttctgcgacaccatgaacagcctgacactgcctagcgaggtgaacctgtgcaatgtggacatcttcaaccccaagtatgattgtaaaatcatgaccagcaagaccgacgtgtccagcagcgtgatcaccagcctgggagccatcgtgagctgctacggcaaaacaaagtgcaccgcctctaacaagaacagaggaattatcaaaaccttcagcaacggctgtgactacgttagcaacaagggagtggatacagtgagcgtgggaaataccctgtactacgtgaacaaacaggaaggcaagtccctgtacgtgaagggcgaacccattatcaacttctacgaccctctggtgttcccaagctgcgagttttgtgccagcatctctcaggtgaacgagaagatcaaccagagcctggccttcatcagaaagagtgatgagctgctgcacaacgtgaacgccgtgaagagcaccacgaatatcatgatcaccaccatcatcatcgtgatcatcgtgatcctgctgagcttaatcgcagttggcctgctcctgtattgttga

SEQ ID NO: 66 - protein, 547 aa, synthetic construct
MELLILKANAITTILTAVTFCFASGQNITEEFYQSTCSAVSKGYLSALRTGWYTSVITIELSNIKKNKCNGTDAKIKLIKQELDKYKNAVTELQLLMGGGSGGGSGGGSGSAIASGVAVCKVLHLEGEVNKIKSALLSTNKAVVSLSNGVSVLTFKVLDLKNYIDKQLLPILNKQSCSISNIETVIEFQQKNNRLLEITREFSVNAGVTTPVSTYMLTNSELLSLINDMPITNDQKKLMSNNVQIVRQQSYSIMCIIKEEVLAYVVQLPLYGVIDTPCWKLHTSPLCTTNTKEGSNICLTRTDRGWYCDNAGSVSFFPQAETCKVQSNRVFCDTMNSLTLPSEVNLCNVDIFNPKYDCKIMTSKTDVSSSVITSLGAIVSCYGKTKCTASNKNRGIIKTFSNGCDYVSNKGVDTVSVGNTLYYVNKQEGKSLYVKGEPIINFYDPLVFPSCEFCASISQVNEKINQSLAFIRKSDELLHNVNAVKSTTNIMITTIIIVIIVILLSLIAVGLLLYCMKQIEDKIEEILSKIYHIENEIARIKKLIGER

SEQ ID NO: 67 - RNA, 1644 nt, synthetic construct
  source 1..1644: mol_type = other RNA
atggaactgctgatcctgaaagccaacgccatcaccaccatcctcaccgccgttaccttctgcttcgcctctggccagaacatcaccgaagagttctaccaaagcacctgcagcgccgtgtccaagggctacctgtctgctctgagaacaggctggtacacaagcgtgatcacaatcgagctgtctaacatcaagaagaacaaatgcaacggcaccgacgccaagattaagctgattaagcaggagctggacaagtacaagaatgccgtgacagagctgcagctgcttatgggcggaggcagcggcggcggctccggtggcggcagcggatctgccatcgcctccggcgtcgccgtgtgcaaggtgctgcacctggaaggcgaggtgaacaagatcaagagcgctctgctcagcacaaacaaggccgtggtgtctctgtccaacggcgtttccgtgctgacctttaaggtgctggacctgaagaattacatcgacaagcagctgctgcctatcctgaacaagcaaagctgtagcatcagcaatattgagacagtgatcgagtttcagcagaagaacaaccggctgctggaaatcacacgggaatttagcgtgaatgccggcgtgaccacacctgtgtctacatacatgctgaccaatagcgagctgctgtctttgatcaacgacatgcctatcacaaatgatcagaaaaagctgatgagcaacaacgtgcaaatcgtgaggcagcagtcatatagcatcatgtgcatcatcaaagaggaagtgctggcctacgtcgtgcagctgccactgtacggcgtcatcgacacaccctgctggaagctgcacacctcccctctgtgcacaaccaacaccaaggaagggtccaacatctgcctgaccagaaccgatagaggctggtactgcgacaatgctggctcagtgagcttcttcccccaggctgaaacctgtaaagtgcagagcaacagagtgttctgcgacaccatgaacagcctgacactgcctagcgaggtgaacctgtgcaatgtggacatcttcaaccccaagtatgattgtaaaatcatgaccagcaagaccgacgtgtccagcagcgtgatcaccagcctgggagccatcgtgagctgctacggcaaaacaaagtgcaccgcctctaacaagaacagaggaattatcaaaaccttcagcaacggctgtgactacgttagcaacaagggagtggatacagtgagcgtgggaaataccctgtactacgtgaacaaacaggaaggcaagtccctgtacgtgaagggcgaacccattatcaacttctacgaccctctggtgttcccaagctgcgagttttgtgccagcatctctcaggtgaacgagaagatcaaccagagcctggccttcatcagaaagagtgatgagctgctgcacaacgtgaacgccgtgaagagcaccacgaatatcatgatcaccaccatcatcatcgtgatcatcgtgatcctgctgagcttaatcgcagttggcctgctcctgtattgtatgaagcagatcgaggacaagatcgaggagatcttgtccaagatctaccacatagagaacgagatagctcggattaagaagctcattggcgagagatga

SEQ ID NO: 68 - protein, 546 aa, synthetic construct
MELLILKANAITTILTAVTFCFASGQNITEEFYQSTCSAVSKGYLSALRTGWYTSVITIELSNIKKNKCNGTDAKIKLIKQELDKYKNAVTELQLLMGGGSGGGSGGGSGSAIASGVAVCKVLHLEGEVNKIKSALLSTNKAVVSLSNGVSVLTFKVLDLKNYIDKQLLPILNKQSCSISNIETVIEFQQKNNRLLEITREFSVNAGVTTPVSTYMLTNSELLSLINDMPITNDQKKLMSNNVQIVRQQSYSIMCIIKEEVLAYVVQLPLYGVIDTPCWKLHTSPLCTTNTKEGSNICLTRTDRGWYCDNAGSVSFFPQAETCKVQSNRVFCDTMNSLTLPSEVNLCNVDIFNPKYDCKIMTSKTDVSSSVITSLGAIVSCYGKTKCTASNKNRGIIKTFSNGCDYVSNKGVDTVSVGNTLYYVNKQEGKSLYVKGEPIINFYDPLVFPSDEFDASISQVNEKINQSLAFIRKSDELLHNVNAVKSTTNIMITTIIIVIIVILLSLIAVGLLLYCSAIGGYIPEAPRDGQAYVRKDGEWVLLSTFL

SEQ ID NO: 69 - RNA, 1641 nt, synthetic construct
  source 1..1641: mol_type = other RNA
atggaactgctgatcctgaaagccaacgccatcaccaccatcctcaccgccgttaccttctgcttcgcctctggccagaacatcaccgaagagttctaccaaagcacctgcagcgccgtgtccaagggctacctgtctgctctgagaacaggctggtacacaagcgtgatcacaatcgagctgtctaacatcaagaagaacaaatgcaacggcaccgacgccaagattaagctgattaagcaggagctggacaagtacaagaatgccgtgacagagctgcagctgcttatgggcggaggcagcggcggcggctccggtggcggcagcggatctgccatcgcctccggcgtcgccgtgtgcaaggtgctgcacctggaaggcgaggtgaacaagatcaagagcgctctgctcagcacaaacaaggccgtggtgtctctgtccaacggcgtttccgtgctgacctttaaggtgctggacctgaagaattacatcgacaagcagctgctgcctatcctgaacaagcaaagctgtagcatcagcaatattgagacagtgatcgagtttcagcagaagaacaaccggctgctggaaatcacacgggaatttagcgtgaatgccggcgtgaccacacctgtgtctacatacatgctgaccaatagcgagctgctgtctttgatcaacgacatgcctatcacaaatgatcagaaaaagctgatgagcaacaacgtgcaaatcgtgaggcagcagtcatatagcatcatgtgcatcatcaaagaggaagtgctggcctacgtcgtgcagctgccactgtacggcgtcatcgacacaccctgctggaagctgcacacctcccctctgtgcacaaccaacaccaaggaagggtccaacatctgcctgaccagaaccgatagaggctggtactgcgacaatgctggctcagtgagcttcttcccccaggctgaaacctgtaaagtgcagagcaacagagtgttctgcgacaccatgaacagcctgacactgcctagcgaggtgaacctgtgcaatgtggacatcttcaaccccaagtatgattgtaaaatcatgaccagcaagaccgacgtgtccagcagcgtgatcaccagcctgggagccatcgtgagctgctacggcaaaacaaagtgcaccgcctctaacaagaacagaggaattatcaaaaccttcagcaacggctgtgactacgttagcaacaagggagtggatacagtgagcgtgggaaataccctgtactacgtgaataaacaggagggcaaatccctgtacgtcaaaggcgagcctatcattaacttctacgaccctctggtgttccccagcgacgagttcgacgcctctatcagccaggtgaacgagaagatcaaccagagcctggccttcatcagaaagtctgatgaactcctgcacaacgtgaacgccgtgaagagcaccaccaacatcatgatcaccaccatcatcatcgtgatcatcgtgatcctgctgagcttaatcgcagttggcctgctcctgtattgttccgctattggcggatacatccctgaggcccctagagatggccaggcctacgtgcggaaggacggcgagtgggtcctgttgtctaccttcctgtga

SEQ ID NO: 70 - protein, 581 aa, synthetic construct
MELLILKANAITTILTAVTFCFASGQNITEEFYQSTCSAVSKGYLSALRTGWYTSVITIELSNIKKNKCNGTDAKIKLIKQELDKYKNAVTELQLLMQSTPATNNRARRELPRFMNYTLNNAKKTNVTLSKKRKRRFLGFLLGVGSAIASGVAVCKVLHLEGEVNKIKSALLSTNKAVVSLSNGVSVLTFKVLDLKNYIDKQLLPILNKQSCSISNIETVIEFQQKNNRLLEITREFSVNAGVTTPVSTYMLTNSELLSLINDMPITNDQKKLMSNNVQIVRQQSYSIMCIIKEEVLAYVVQLPLYGVIDTPCWKLHTSPLCTTNTKEGSNICLTRTDRGWYCDNAGSVSFFPQAETCKVQSNRVFCDTMNSLTLPSEVNLCNVDIFNPKYDCKIMTSKTDVSSSVITSLGAIVSCYGKTKCTASNKNRGIIKTFSNGCDYVSNKGVDTVSVGNTLYYVNKQEGKSLYVKGEPIINFYDPLVFPSDEFDASISQVNEKINQSLAFIRKSDELLHNVNAVKSTTNIMITTIIIVIIVILLSLIAVGLLLYCSAIGGYIPEAPRDGQAYVRKDGEWVLLSTFL

SEQ ID NO: 71 - RNA, 1746 nt, synthetic construct
  source 1..1746: mol_type = other RNA
atggaactgctgatcctgaaagccaacgccatcaccaccatcctcaccgccgttaccttctgcttcgcctctggccagaacatcaccgaagagttctaccaaagcacctgcagcgccgtgtccaagggctacctgtctgctctgagaacaggctggtacacaagcgtgatcacaatcgagctgtctaacatcaagaagaacaaatgcaacggcaccgacgccaagattaagctgattaagcaggagctggacaagtacaagaatgccgtgacagagctgcagctgcttatgcagagcacccctgccaccaacaacagagccaggcgggaactgcctagattcatgaactacaccctgaacaatgctaaaaagaccaatgtgacactgagcaagaagcggaaaagacggttcctgggatttctgctgggcgtcggatctgccatcgcctccggcgtcgccgtgtgcaaggtgctgcacctggaaggcgaggtgaacaagatcaagagcgctctgctcagcacaaacaaggccgtggtgtctctgtccaacggcgtttccgtgctgacctttaaggtgctggacctgaagaattacatcgacaagcagctgctgcctatcctgaacaagcaaagctgtagcatcagcaatattgagacagtgatcgagtttcagcagaagaacaaccggctgctggaaatcacacgggaatttagcgtgaatgccggcgtgaccacacctgtgtctacatacatgctgaccaatagcgagctgctgtctttgatcaacgacatgcctatcacaaatgatcagaaaaagctgatgagcaacaacgtgcaaatcgtgaggcagcagtcatatagcatcatgtgcatcatcaaagaggaagtgctggcctacgtcgtgcagctgccactgtacggcgtcatcgacacaccctgctggaagctgcacacctcccctctgtgcacaaccaacaccaaggaagggtccaacatctgcctgaccagaaccgatagaggctggtactgcgacaatgctggctcagtgagcttcttcccccaggctgaaacctgtaaagtgcagagcaacagagtgttctgcgacaccatgaacagcctgacactgcctagcgaggtgaacctgtgcaatgtggacatcttcaaccccaagtatgattgtaaaatcatgaccagcaagaccgacgtgtccagcagcgtgatcaccagcctgggagccatcgtgagctgctacggcaaaacaaagtgcaccgcctctaacaagaacagaggaattatcaaaaccttcagcaacggctgtgactacgttagcaacaagggagtggatacagtgagcgtgggaaataccctgtactacgtgaataaacaggagggcaaatccctgtacgtcaaaggcgagcctatcattaacttctacgaccctctggtgttccccagcgacgagttcgacgcctctatcagccaggtgaacgagaagatcaaccagagcctggccttcatcagaaagtctgatgaactcctgcacaacgtgaacgccgtgaagagcaccaccaacatcatgatcaccaccatcatcatcgtgatcatcgtgatcctgctgagcttaatcgcagttggcctgctcctgtattgttccgctattggcggatacatccctgaggcccctagagatggccaggcctacgtgcggaaggacggcgagtgggtcctgttgtctaccttcctgtga

SEQ ID NO: 72 - protein, 581 aa, synthetic construct
MELLILKANAITTILTAVTFCFASGQNITEEFYQSTCSAVSKGYLSALRTGWYTSVITIELSNIKKNKCNGTDAKIKLIKQELDKYKNAVTELQLLMQSTPATNNRARRELPRFMNYTLNNAKKTNVTLSKKRKRRFLGFLLGVGSAIASGVAVCKVLHLEGEVNKIKSALLSTNKAVVSLSNGVSVLTFKVLDLKNYIDKQLLPILNKQSCSISNIETVIEFQQKNNRLLEITREFSVNAGVTTPVSTYMLTNSELLSLINDMPITNDQKKLMSNNVQIVRQQSYSIMCIIKEEVLAYVVQLPLYGVIDTPCWKLHTSPLCTTNTKEGSNICLTRTDRGWYCDNAGSVSFFPQAETCKVQSNRVFCDTMNSLTLPSEVNLCNVDIFNPKYDCKIMTSKTDVSSSVITSLGAIVSCYGKTKCTASNKNRGIIKTFSNGCDYVSNKGVDTVSVGNTLYYVNKQEGKSLYVKGEPIINFYDPLVFPSCEFCASISQVNEKINQSLAFIRKSDELLHNVNAVKSTTNIMITTIIIVIIVILLSLIAVGLLLYCSAIGGYIPEAPRDGQAYVRKDGEWVLLSTFL

SEQ ID NO: 73 - RNA, 1746 nt, synthetic construct
  source 1..1746: mol_type = other RNA
atggaactgctgatcctgaaagccaacgccatcaccaccatcctcaccgccgttaccttctgcttcgcctctggccagaacatcaccgaagagttctaccaaagcacctgcagcgccgtgtccaagggctacctgtctgctctgagaacaggctggtacacaagcgtgatcacaatcgagctgtctaacatcaagaagaacaaatgcaacggcaccgacgccaagattaagctgattaagcaggagctggacaagtacaagaatgccgtgacagagctgcagctgcttatgcagagcacccctgccaccaacaacagagccaggcgggaactgcctagattcatgaactacaccctgaacaatgctaaaaagaccaatgtgacactgagcaagaagcggaaaagacggttcctgggatttctgctgggcgtcggatctgccatcgcctccggcgtcgccgtgtgcaaggtgctgcacctggaaggcgaggtgaacaagatcaagagcgctctgctcagcacaaacaaggccgtggtgtctctgtccaacggcgtttccgtgctgacctttaaggtgctggacctgaagaattacatcgacaagcagctgctgcctatcctgaacaagcaaagctgtagcatcagcaatattgagacagtgatcgagtttcagcagaagaacaaccggctgctggaaatcacacgggaatttagcgtgaatgccggcgtgaccacacctgtgtctacatacatgctgaccaatagcgagctgctgtctttgatcaacgacatgcctatcacaaatgatcagaaaaagctgatgagcaacaacgtgcaaatcgtgaggcagcagtcatatagcatcatgtgcatcatcaaagaggaagtgctggcctacgtcgtgcagctgccactgtacggcgtcatcgacacaccctgctggaagctgcacacctcccctctgtgcacaaccaacaccaaggaagggtccaacatctgcctgaccagaaccgatagaggctggtactgcgacaatgctggctcagtgagcttcttcccccaggctgaaacctgtaaagtgcagagcaacagagtgttctgcgacaccatgaacagcctgacactgcctagcgaggtgaacctgtgcaatgtggacatcttcaaccccaagtatgattgtaaaatcatgaccagcaagaccgacgtgtccagcagcgtgatcaccagcctgggagccatcgtgagctgctacggcaaaacaaagtgcaccgcctctaacaagaacagaggaattatcaaaaccttcagcaacggctgtgactacgttagcaacaagggagtggatacagtgagcgtgggaaataccctgtactacgtgaacaaacaggaaggcaagtccctgtacgtgaagggcgaacccattatcaacttctacgaccctctggtgttcccaagctgcgagttttgtgccagcatctctcaggtgaacgagaagatcaaccagagcctggccttcatcagaaagagtgatgagctgctgcacaacgtgaacgccgtgaagagcaccacgaatatcatgatcaccaccatcatcatcgtgatcatcgtgatcctgctgagcttaatcgcagttggcctgctcctgtattgttccgctattggcggatacatccctgaggcccctagagatggccaggcctacgtgcggaaggacggcgagtgggtcctgttgtctaccttcctgtga

SEQ ID NO: 74 - protein, 12 aa, synthetic construct
GGGSGGGSGGGS

SEQ ID NO: 75 - RNA, 36 nt, synthetic construct
  source 1..36: mol_type = other RNA
ggcggaggcagcggcggcggctccggtggcggcagc

SEQ ID NO: 76 - protein, 566 aa, synthetic construct
MELLILKANAITTILTAVTFCFASGQNITEEFYQSTCSAVSKGYLSALRTGWYTSVITIELSNIKKNKCNGTDAKIKLIKQELDKYKNAVTELQLLMQSTPATNNRARRGGGSGGGSGGGSFLGFLLGVGSAIASGVAVCKVLHLEGEVNKIKSALLSTNKAVVSLSNGVSVLTFKVLDLKNYIDKQLLPILNKQSCSISNIETVIEFQQKNNRLLEITREFSVNAGVTTPVSTYMLTNSELLSLINDMPITNDQKKLMSNNVQIVRQQSYSIMCIIKEEVLAYVVQLPLYGVIDTPCWKLHTSPLCTTNTKEGSNICLTRTDRGWYCDNAGSVSFFPQAETCKVQSNRVFCDTMNSLTLPSEVNLCNVDIFNPKYDCKIMTSKTDVSSSVITSLGAIVSCYGKTKCTASNKNRGIIKTFSNGCDYVSNKGVDTVSVGNTLYYVNKQEGKSLYVKGEPIINFYDPLVFPSCEFCASISQVNEKINQSLAFIRKSDELLHNVNAVKSTTNIMITTIIIVIIVILLSLIAVGLLLYCSAIGGYIPEAPRDGQAYVRKDGEWVLLSTFL

SEQ ID NO: 77 - RNA, 1701 nt, synthetic construct
  source 1..1701: mol_type = other RNA
atggaactgctgatcctgaaagccaacgccatcaccaccatcctcaccgccgttaccttctgcttcgcctctggccagaacatcaccgaagagttctaccaaagcacctgcagcgccgtgtccaagggctacctgtctgctctgagaacaggctggtacacaagcgtgatcacaatcgagctgtctaacatcaagaagaacaaatgcaacggcaccgacgccaagattaagctgattaagcaggagctggacaagtacaagaatgccgtgacagagctgcagctgcttatgcagagcacccctgccaccaacaacagagccaggcggggcggaggcagcggcggcggctccggtggcggcagcttcctgggatttctgctgggcgtcggatctgccatcgcctccggcgtcgccgtgtgcaaggtgctgcacctggaaggcgaggtgaacaagatcaagagcgctctgctcagcacaaacaaggccgtggtgtctctgtccaacggcgtttccgtgctgacctttaaggtgctggacctgaagaattacatcgacaagcagctgctgcctatcctgaacaagcaaagctgtagcatcagcaatattgagacagtgatcgagtttcagcagaagaacaaccggctgctggaaatcacacgggaatttagcgtgaatgccggcgtgaccacacctgtgtctacatacatgctgaccaatagcgagctgctgtctttgatcaacgacatgcctatcacaaatgatcagaaaaagctgatgagcaacaacgtgcaaatcgtgaggcagcagtcatatagcatcatgtgcatcatcaaagaggaagtgctggcctacgtcgtgcagctgccactgtacggcgtcatcgacacaccctgctggaagctgcacacctcccctctgtgcacaaccaacaccaaggaagggtccaacatctgcctgaccagaaccgatagaggctggtactgcgacaatgctggctcagtgagcttcttcccccaggctgaaacctgtaaagtgcagagcaacagagtgttctgcgacaccatgaacagcctgacactgcctagcgaggtgaacctgtgcaatgtggacatcttcaaccccaagtatgattgtaaaatcatgaccagcaagaccgacgtgtccagcagcgtgatcaccagcctgggagccatcgtgagctgctacggcaaaacaaagtgcaccgcctctaacaagaacagaggaattatcaaaaccttcagcaacggctgtgactacgttagcaacaagggagtggatacagtgagcgtgggaaataccctgtactacgtgaacaaacaggaaggcaagtccctgtacgtgaagggcgaacccattatcaacttctacgaccctctggtgttcccaagctgcgagttttgtgccagcatctctcaggtgaacgagaagatcaaccagagcctggccttcatcagaaagagtgatgagctgctgcacaacgtgaacgccgtgaagagcaccacgaatatcatgatcaccaccatcatcatcgtgatcatcgtgatcctgctgagcttaatcgcagttggcctgctcctgtattgttccgctattggcggatacatccctgaggcccctagagatggccaggcctacgtgcggaaggacggcgagtgggtcctgttgtctaccttcctgtga

SEQ ID NO: 78 - protein, 530 aa, synthetic construct
MELLILKANAITTILTAVTFCFASGQNITEEFYQSTCSAVSKGYLSALRTGWYTSVITIELSNIKKNKCNGTDAKIKLIKQELDKYKNAVTELQLLMGGGSGGGSGGGSGSAIASGVAVCKVLHLEGEVNKIKSALLSTNKAVVSLSNGVSVLTFKVLDLKNYIDKQLLPILNKQSCSISNIETVIEFQQKNNRLLEITREFSVNAGVTTPVSTYMLTNSELLSLINDMPITNDQKKLMSNNVQIVRQQSYSIMCIIKEEVLAYVVQLPLYGVIDTPCWKLHTSPLCTTNTKEGSNICLTRTDRGWYCDNAGSVSFFPQAETCKVQSNRVFCDTMNSLTLPSEVNLCNVDIFNPKYDCKIMTSKTDVSSSVITSLGAIVSCYGKTKCTASNKNRGIIKTFSNGCDYVSNKGVDTVSVGNTLYYVNKQEGKSLYVKGEPIINFYDPLVFPSCEFCASISQVNEKINQSLAFIRKSDELLIIIVIIVILLSLIAVGLLLYCSAIGGYIPEAPRDGQAYVRKDGEWVLLSTFL

SEQ ID NO: 79 - RNA, 1593 nt, synthetic construct
  source 1..1593: mol_type = other RNA
atggaactgctgatcctgaaagccaacgccatcaccaccatcctcaccgccgttaccttctgcttcgcctctggccagaacatcaccgaagagttctaccaaagcacctgcagcgccgtgtccaagggctacctgtctgctctgagaacaggctggtacacaagcgtgatcacaatcgagctgtctaacatcaagaagaacaaatgcaacggcaccgacgccaagattaagctgattaagcaggagctggacaagtacaagaatgccgtgacagagctgcagctgcttatgggcggaggcagcggcggcggctccggtggcggcagcggatctgccatcgcctccggcgtcgccgtgtgcaaggtgctgcacctggaaggcgaggtgaacaagatcaagagcgctctgctcagcacaaacaaggccgtggtgtctctgtccaacggcgtttccgtgctgacctttaaggtgctggacctgaagaattacatcgacaagcagctgctgcctatcctgaacaagcaaagctgtagcatcagcaatattgagacagtgatcgagtttcagcagaagaacaaccggctgctggaaatcacacgggaatttagcgtgaatgccggcgtgaccacacctgtgtctacatacatgctgaccaatagcgagctgctgtctttgatcaacgacatgcctatcacaaatgatcagaaaaagctgatgagcaacaacgtgcaaatcgtgaggcagcagtcatatagcatcatgtgcatcatcaaagaggaagtgctggcctacgtcgtgcagctgccactgtacggcgtcatcgacacaccctgctggaagctgcacacctcccctctgtgcacaaccaacaccaaggaagggtccaacatctgcctgaccagaaccgatagaggctggtactgcgacaatgctggctcagtgagcttcttcccccaggctgaaacctgtaaagtgcagagcaacagagtgttctgcgacaccatgaacagcctgacactgcctagcgaggtgaacctgtgcaatgtggacatcttcaaccccaagtatgattgtaaaatcatgaccagcaagaccgacgtgtccagcagcgtgatcaccagcctgggagccatcgtgagctgctacggcaaaacaaagtgcaccgcctctaacaagaacagaggaattatcaaaaccttcagcaacggctgtgactacgttagcaacaagggagtggatacagtgagcgtgggaaataccctgtactacgtgaacaaacaggaaggcaagtccctgtacgtgaagggcgaacccattatcaacttctacgaccctctggtgttcccaagctgcgagttttgtgccagcatctctcaggtgaacgagaagatcaaccagagcctggccttcatcagaaagagtgatgagctgctgatcatcatcgtgatcatcgtgatcctgctgagcttaatcgcagttggcctgctcctgtattgttccgctattggcggatacatccctgaggcccctagagatggccaggcctacgtgcggaaggacggcgagtgggtcctgttgtctaccttcctgtga

SEQ ID NO: 80 - protein, 526 aa, synthetic construct; identical to SEQ ID NO: 28

SEQ ID NO: 81 - RNA, 1581 nt, synthetic construct; identical to SEQ ID NO: 29
  source 1..1581: mol_type = other RNA

SEQ ID NO: 82 - protein, 535 aa, synthetic construct; identical to SEQ ID NO: 30

SEQ ID NO: 83 - RNA, 1608 nt, synthetic construct; identical to SEQ ID NO: 31
  source 1..1608: mol_type = other RNA

SEQ ID NO: 84 - RNA, 1641 nt, synthetic construct
  source 1..1641: mol_type = other RNA
atggaactcctgatcctgaaagccaacgccatcacaaccatcctgaccgccgttaccttctgcttcgccagcggacagaacattacagaggaattctaccagagcacatgtagcgctgtgtctaaaggctacctgagcgccctgcggaccggatggtacaccagtgtgatcaccatcgagctgagtaatatcaagaagaacaaatgcaacgggaccgacgccaagatcaaactgatcaagcaggagctggataagtacaagaatgccgtgaccgagctgcagctgctgatgggcggcggaagcggcggcggctctggcggaggctcaggctctgctatcgcctccggagtcgccgtctgcaaagtcctgcacctggaaggcgaggtgaacaagatcaagtctgccctgctgagcaccaacaaggccgtggtgtctttaagcaatggcgtgagcgtgctgacattcaaggtgctggacctgaagaactacattgataagcagctgctgcctatcctgaacaagcagagctgtagcatctccaacatcgaaaccgttatcgaatttcagcaaaagaacaatagactgcttgagatcacaagagagttcagcgtgaatgccggagtaacaacacccgtgtccacatacatgctgaccaactctgaactgctatccctgatcaacgacatgcctatcaccaatgaccagaagaaactgatgagcaacaacgtgcaaatcgtgagacagcagagctacagcatcatgtgcatcatcaaggaagaggtgctggcttacgtggtgcagctgcccctgtacggcgtgatcgacaccccttgctggaagctgcacacatctccactctgtaccaccaacacaaaggaaggcagcaatatttgtctgactcggaccgatagaggctggtattgtgataacgcgggcagcgtgtccttcttcccccaggccgagacatgcaaggtgcagagcaatagagtgttctgcgacacaatgaacagcctcaccctgcctagcgaggtgaacctgtgcaatgtggacatcttcaaccccaagtacgactgcaagatcatgaccagcaagaccgacgtgtccagcagcgtgatcaccagcctgggagccatcgtgagctgctacggcaagaccaagtgcaccgcctctaataaaaaccggggcatcatcaagacattcagcaacggttgtgactacgtgagcaacaagggcgtggacaccgtgtccgtcggcaacaccctgtactacgtgaacaaacaagagggcaaaagcctgtacgtgaagggcgagcctatcatcaacttctacgatcctctggtctttccatcttgcgagttttgcgcctccatcagccaggtgaacgagaagatcaaccagagcctggccttcatcagaaagagcgacgagctgctgcacaacgtgaacgctgtgaagagcaccacaaacatcatgatcactaccatcatcatcgtgatcattgttatcctgctgagcctgatcgccgtgggcctgctgctgtattgcagcgctattggcggctatatccctgaggcccctagagatggccaggcctacgtgcggaaggacggcgaatgggtgctgctgtctacctttctgtga

SEQ ID NO: 85 - RNA, 1641 nt, synthetic construct
  source 1..1641: mol_type = other RNA
atggaactgctgatcctcaaggccaacgctattaccacaatcctgacagccgtgaccttctgcttcgccagcggccagaacatcaccgaggaattttaccagagcacatgcagcgccgtttccaagggatatctgagcgctctgagaacaggctggtatacatctgttatcaccatcgagctgagcaacatcaagaagaacaagtgtaatggcaccgatgccaagatcaaactgatcaaacaggagctggataagtacaagaacgccgtgaccgagctgcagctgctgatgggcggaggctccggcggcggcagtggcggaggaagcggcagcgccatcgcctccggcgtggctgtgtgcaaagtgctgcacctggaaggcgaggtgaacaagatcaagtccgcactgctgtctacaaacaaagctgtggtgagcctgagcaatggcgtctccgtgctgaccttcaaggtgctcgacctgaaaaactacatcgacaagcagctgctgccaatcctgaacaagcagagctgcagcatcagcaacatcgagacagtgatcgagtttcagcaaaagaacaacaggctgctggaaatcacccgggaattcagcgtgaacgccggcgtcacaacccctgtgtctacatacatgctcaccaattccgagctgctgtctctgatcaacgacatgcctatcacaaatgatcagaaaaagctgatgagcaacaatgtgcaaatcgtgcggcagcagagctacagcatcatgtgcatcatcaaggaggaagtgctggcctacgtggtgcagctgcctctgtacggtgtgattgacaccccttgttggaagctgcacacctcccctctgtgcaccacaaataccaaggaaggcagcaacatctgtctgacaagaaccgatagaggatggtactgcgacaacgccggcagcgtgagcttcttcccacaggctgaaacctgcaaggtgcagtctaatagagtgttctgtgataccatgaacagcctgaccctgcctagcgaggtgaacctgtgcaacgtcgacatcttcaaccccaagtacgactgcaagattatgaccagcaagaccgacgtgtcttctagcgtgatcacctccctgggagccatcgtcagctgctacggcaagacaaagtgcaccgccagcaacaagaaccgcggcatcatcaaaacctttagcaatggatgtgactacgtgtctaacaaaggcgtggacaccgtgagcgtgggcaacaccctgtactacgtgaacaagcaagagggcaagtccctgtacgttaagggcgagcctatcatcaacttctacgaccccctggtgttccccagctgtgaattctgcgcctctatctctcaggtgaacgagaagattaaccagtccctggcctttatcagaaagagcgacgagctgctgcacaacgtgaatgccgtcaagtctacaaccaacatcatgatcaccacgattatcatcgtgatcatcgtgatcctgctgtctctgatcgccgttggactgctgctctattgcagcgccatcggcggctacatccccgaggcccctagagatggccaggcctacgtgcggaaggacggcgaatgggtgctgctaagcaccttcctgtga

SEQ ID NO: 86 - RNA, 1641 nt, synthetic construct
  source 1..1641: mol_type = other RNA
atggaactgcttattctgaaggctaacgccatcaccaccatcctgactgccgtcaccttttgcttcgccagcggacagaacatcaccgaggaattttaccagagcacctgttccgccgtgagcaagggctacctgagcgctctgagaaccggctggtacaccagcgtgatcacaatcgagctcagcaacatcaagaagaacaagtgcaacggcaccgacgccaagatcaaactgatcaagcaggagctggataagtacaagaatgccgtgacagagctgcagctgctgatgggcggcggcagcggcggcggatctggcggcggttctggctctgctatcgctagcggcgttgctgtgtgcaaagtgctgcacctggaaggcgaggtgaacaagatcaagagcgccctgctgtcgaccaacaaagccgtggtgagtctctccaatggcgtgagcgtgctgaccttcaaggtgctggacctgaaaaattacatcgacaagcagctgctgcctatcctgaacaagcagagctgtagcatcagcaacatcgagaccgtgatagagttccagcagaagaacaaccggctgctggaaatcacacgggaattcagcgtgaacgccggagtgaccacacctgtgtccacatacatgctgacaaactccgagctgctgtctctgatcaacgacatgcctattaccaacgaccagaaaaagctgatgagcaataacgtgcagatcgtgcggcagcaaagctactccatcatgtgcatcatcaaagaggaagtcctggcctacgtggtgcaactgcctctgtacggcgtgattgacaccccttgttggaagctgcacaccagcccactgtgcacaaccaacaccaaggaaggctctaatatctgcctaacaagaacagatagaggctggtattgtgacaacgccggctctgtgagcttcttccctcaggccgagacatgcaaggtgcaaagcaacagagtgttctgtgataccatgaacagcctgaccctaccatctgaagtgaacctgtgtaacgttgacatcttcaaccccaaatacgactgcaagatcatgaccagcaagaccgatgtgtcatccagcgttatcaccagcctgggcgccatcgtgagctgctacggaaagaccaagtgcaccgccagcaacaagaacagaggaatcatcaagacattcagcaatggctgcgattacgtgtctaacaagggcgtggacacagtgtccgtgggaaataccctgtactacgtgaacaaacaggagggcaaaagcctgtacgtgaagggcgaacctatcattaacttctacgaccccctggtgttccccagctgcgagttttgcgccagcatctctcaggtgaacgagaagatcaaccagtctctggctttcatcagaaagagcgacgagctgctccacaacgtgaatgccgtcaagagcactacaaacatcatgatcaccaccatcatcatcgtgatcatcgtgatcctgctgagcctgatcgccgtgggcctgctgctgtattgcagcgccatcggcggatacatccccgaggcccctagggatggccaggcttatgtcagaaaggacggagaatgggtgctgctgagcacattcctgtga

SEQ ID NO: 87 - RNA, 1641 nt, synthetic construct
  source 1..1641: mol_type = other RNA
atggaactgctgattctgaaggctaatgctatcactaccatcctgaccgccgtgaccttctgcttcgccagcggccagaacatcaccgaggaattttaccagtccacatgtagcgcggtgagcaagggttatctgagcgccctgagaacaggctggtacacctccgtcatcaccatcgaactgagcaacatcaagaagaacaagtgcaatggcaccgatgccaagatcaagctgatcaaacaggagctggataagtacaagaacgccgtgaccgaactgcagctgctgatgggcggcggcagtggaggcggcagcggcggaggctccggcagcgctatcgccagcggcgtggccgtgtgcaaggtgctgcacctggaaggcgaggtgaacaaaatcaagagcgccctgctgagcacaaataaggccgttgtgtcactgagcaacggagtgagcgtgctcaccttcaaggtcctggacctgaaaaattacatcgacaagcaattactgcctatcctgaacaagcagagctgtagcatcagcaatatcgagaccgttatcgagttccagcagaaaaacaacagactgctggaaatcactcgggaattcagcgtgaacgccggcgtgacaacccctgtgagcacctacatgctgaccaacagcgagctcctgtctctgattaacgacatgcctatcaccaatgaccagaagaaactaatgagcaacaacgtgcagatcgtgcggcagcaatcctacagcatcatgtgcatcatcaaggaagaggtgctggcctacgtggtgcagctgcctctgtacggagtgattgataccccatgttggaagctgcacaccagccctctgtgcacaaccaataccaaagaaggctctaatatctgcctgaccagaaccgacaggggctggtattgcgacaacgctggcagcgtgagcttcttcccccaggccgagacctgtaaagtgcagagcaacagagtgttctgcgacaccatgaactccctgacactgcccagcgaggtgaacctgtgtaacgtggatatcttcaaccccaagtacgactgcaagatcatgacctctaagaccgacgtgtctagcagcgtgatcaccagcctgggcgccatcgtgtcttgctacggcaaaaccaaatgcaccgccagcaacaagaaccggggcatcatcaagacctttagcaacggctgcgattacgtgtctaacaaaggcgtggacacagtgtctgtcggaaataccctgtactacgtgaacaagcaagagggcaagtctctctacgttaagggcgagcctatcatcaacttctacgaccctctggtgttcccatcatgcgagttttgtgcctctatctcccaggtgaacgagaagatcaaccagtccctggccttcatcagaaagagcgacgagctgctgcacaacgtgaacgccgttaagagcacaacaaatatcatgattacaacaatcatcatcgtcatcatcgtgatcctgctgtccctcatcgccgtgggcctgctgctgtactgcagcgccataggaggatatatccccgaggcccctagagatggacaggcttacgtgagaaaggacggcgaatgggtgctgctgtctacatttctgtga

SEQ ID NO: 88 - RNA, 1644 nt, synthetic construct
  source 1..1644: mol_type = other RNA
atggaactgctgatcctcaaggccaacgctatcaccacaatcctgacagctgttaccttttgcttcgccagcggccagaacatcaccgaggaattctaccagagcacctgtagcgctgtgagcaagggctacctgagcgccctgagaaccggctggtacacctctgttatcacaatcgagctgtctaacattaagaaaaacaagtgcaatggaacagacgccaagatcaaactgatcaagcaagagctggataagtacaagaacgccgtgacagagctgcagttactgatgggcggaggcagcggcggaggcagcggcggcggctctggctctgccatcgcctctggtgtcgccgtgtgcaaagtgctgcatctggaaggcgaagtgaacaaaatcaagtccgccctgctgagcaccaacaaagccgtggtgtccctgagcaatggcgtgagcgtgctgacatttaaggtgctggacctgaagaactacatcgacaagcagctgctgcccatcctgaataagcagtcttgctctattagcaacatcgaaaccgtgatcgagttccagcagaaaaacaacaggctgctcgagatcaccagagagtttagcgtgaacgccggcgtgaccacccctgtctccacctacatgctgacaaattccgagctgctgagcctgatcaatgacatgcctatcacaaacgaccagaagaagctgatgagcaacaatgtgcaaatcgttagacagcagagctacagcatcatgtgcatcatcaaggaagaagtgcttgcttatgtggtgcagctgccactgtacggcgtgatcgatacaccttgctggaagctgcacaccagccctctgtgcaccaccaacaccaaggaaggcagcaatatctgcctgacccggaccgatagaggctggtattgtgacaacgctggcagcgtgagcttcttcccccaggccgagacatgcaaggtgcagagtaacagagtgttctgtgataccatgaacagcctgaccctgcctagcgaagtgaacctgtgcaacgtggacatcttcaaccccaagtacgactgcaagatcatgaccagcaagaccgacgtgagttctagcgtgatcaccagcctgggcgccatcgtgagctgctacggcaaaaccaagtgtacagccagcaacaagaaccggggcatcatcaagaccttcagcaacggctgcgactacgtgagcaacaagggagtcgataccgtgtcagtgggaaataccctgtactacgtcaataagcaggagggcaagtcgctgtacgtgaagggcgagcctatcatcaacttctatgatcctctggtgttcccatcttgtgagttctgcgcctccatcagccaggtgaatgagaaaatcaaccagagcctggccttcatcagaaagagcgacgagctgctgcacaacgtgaacgccgtgaagtccacaacaaacatcatgatcaccacaatcatcattgtgatcattgtaatcctgctcagcctgatcgccgtgggcctgctgctgtactgtatgaaacaaatcgaggacaagatcgaggaaatcctgtccaagatctaccacatcgagaacgagatcgccagaatcaagaaactgataggagaacggtga

SEQ ID NO: 89 - RNA, 1644 nt, synthetic construct
  source 1..1644: mol_type = other RNA
atggaactgctgatcctgaaggccaacgctatcacaacaatcctgaccgccgtgacattctgcttcgccagcggccagaacatcaccgaggaattctaccagagcacatgcagcgctgtgtcaaagggttatctgagcgccctgagaacaggctggtacacctctgtgattacaatcgagctgagcaacatcaagaagaacaagtgcaacggcaccgacgccaagatcaagttaattaagcaagagctcgacaagtacaagaatgccgtgacggaactgcagctgctcatgggcggcggaagcggcggaggaagcggaggcggaagcggctctgccattgcctctggcgtggccgtttgtaaagtgctgcacctggaaggcgaagtgaacaagatcaagagcgccctattgagcaccaacaaggccgtcgtctctctgtccaatggcgttagcgtgctgaccttcaaggtgctggatctgaagaactacatcgacaagcaactgctgcctatcctgaacaaacagtcttgttctatcagcaacatcgaaaccgtgatcgagttccagcagaagaacaaccggctgctggaaattacccgggaattttctgtgaacgccggcgtgaccacccctgtgtccacctacatgctgacaaatagcgagctgctgtctctgatcaacgacatgcctatcaccaatgaccagaaaaagctgatgagcaacaacgtgcaaatcgttagacagcagagctacagcatcatgtgcatcatcaaggaagaggtgctggcctacgtggtgcagctgcctctgtacggcgtgatcgacaccccatgttggaagctgcacaccagccccctgtgcaccacaaacaccaaagaaggaagcaatatctgcctgacacggaccgatagaggctggtattgcgacaacgctggcagcgtgtccttcttccctcaggccgagacatgtaaagtgcagagcaacagagtgttctgcgacaccatgaacagcctgacactgcctagcgaggtgaacctgtgtaatgtcgacatcttcaaccccaagtacgactgcaagatcatgaccagcaagacagacgtgtctagcagcgtgatcacctccctgggcgctatcgtgagctgctacggcaagaccaagtgtaccgccagtaataaaaatcgcggcatcattaaaactttcagcaatggctgcgattacgtgtccaacaagggcgttgatacagtgtctgtcggcaacaccctgtattacgtgaacaaacaggagggcaagagcctgtacgtgaaaggcgagcccattatcaacttctacgaccccctggtgtttccttcttgcgagttttgcgccagcatcagccaggtgaacgagaagatcaaccagtccctcgccttcatcagaaagtccgatgagctgctgcataacgtgaacgccgtgaagtctacaaccaacatcatgatcaccaccatcatcatcgtgatcatcgtgatcctgctgtctctgatcgccgtgggcctgctgctgtactgcatgaagcagatcgaagataagatcgaggaaatcctgagcaaaatctaccacatcgagaacgagatcgccagaatcaagaagctgatcggcgagagatga

SEQ ID NO: 90 - RNA, 1644 nt, synthetic construct
  source 1..1644: mol_type = other RNA
atggaactgctgatcctgaaggccaacgctattaccaccatcctgacggccgtgacattttgcttcgcctctggccagaacatcacagaagagttctaccagagcacatgtagcgccgtgtccaaaggctacctgagcgccctgaggaccggctggtacaccagcgtgatcacaatcgagctttctaacatcaagaagaacaaatgcaacggcaccgatgccaagattaagctcatcaagcaagagctggacaagtacaagaacgccgtcacagagctgcagctgctgatgggcggcggatctggaggaggctctggcggcggcagcggctctgctatcgccagcggcgtggccgtgtgcaaggtgctgcatctggaaggcgaggtgaataaaattaagagcgccctgctgtcaacaaacaaagccgtggtgagcctgagcaatggcgtgtctgtgctgaccttcaaggtgctggatctgaaaaactacatcgacaagcagctgctgcctatcctcaacaagcagtcctgttctattagcaacatcgagacagtgatcgaatttcagcagaagaacaatcggctgctggaaatcacaagagagttcagcgtgaacgctggagtgaccacacctgtgagcacctatatgctgacaaacagcgagctgctgtctctgatcaacgacatgcctatcacaaacgaccagaagaagctgatgagcaacaacgttcagatcgtgcggcagcaaagctacagcatcatgtgcatcatcaaggaagaagtgctcgcctacgtggtgcagctgcctctgtacggcgtgatcgacaccccttgctggaaactgcacaccagccccctgtgcaccaccaataccaaggaaggcagcaatatctgcctgaccagaaccgatagaggatggtattgtgacaacgccggcagcgtgtccttcttcccccaggccgagacctgcaaggtgcagagcaacagagtgttctgcgacaccatgaactccctgaccctgccaagcgaggtgaacctgtgtaatgtggacatcttcaaccccaagtatgactgcaagatcatgaccagcaagacggacgtgtccagcagcgtaattacaagcttaggcgccatcgtgtcatgttacggcaagaccaaatgtaccgccagcaataaaaaccggggcatcatcaaaacctttagcaacggctgcgactacgtcagcaataagggcgttgataccgtgagcgtgggaaataccctgtactacgtgaacaagcaggagggcaagtccctgtacgtgaagggcgagcctatcatcaacttctacgaccccctggtcttccctagctgcgagttctgcgccagcatcagccaggtgaatgagaagattaaccagagcctggccttcatcagaaagagcgatgagctgctgcacaacgtcaacgctgtcaagtctaccacaaacatcatgatcacaaccatcatcatcgtgatcatagttatcctgctgtccctgatcgctgtgggactgctgctgtactgcatgaaacaaatcgaagataagatcgaggaaatcctgagtaagatctaccacatcgagaacgagatcgcccggatcaagaaactgatcggcgaaagatga

SEQ ID NO: 91 - RNA, 1644 nt, synthetic construct
  source 1..1644: mol_type = other RNA
atggaactgctcatcctgaaggccaacgctatcacaaccatcctgacggccgtgaccttttgcttcgccagcggccagaacatcaccgaagaattctaccaatctacctgtagcgccgtgtccaagggctacctgtctgccctgagaaccggctggtacacatctgtgatcaccatcgagctgagcaacatcaaaaagaacaagtgcaacggaacagacgccaagatcaaactgattaaacaagagctggacaagtacaagaacgctgtgacagagctgcagctgctgatgggcggcggcagcggcggaggcagcggaggcggaagcggcagcgccatcgccagcggcgtcgccgtgtgcaaggtgctgcatctggaaggagaagtgaacaagatcaagtctgctctgctgagcaccaacaaagccgtggtgtccctgtctaatggcgtgtccgtgctgaccttcaaggtgctggatctgaagaattacatcgacaagcagctgctccccatcctgaacaagcaaagctgcagtatcagcaatattgagacagtgattgaatttcagcagaagaacaaccggctgcttgagatcacccgcgagttttccgttaatgctggcgtgaccacacctgtgtctacatacatgctgaccaacagcgagctgctgtccctgatcaacgacatgcctatcaccaatgatcagaaaaagctgatgagtaacaacgtacagatcgtgcggcagcagagctacagcatcatgtgcatcatcaaggaagaggtgctggcctacgtggtccagctgcctctgtacggcgtgatcgacacaccatgttggaagctgcacaccagccctctgtgtaccacaaataccaaggaaggcagcaatatctgcctgaccagaacagatagaggctggtattgtgacaacgccggctctgtgagcttcttcccccaggccgaaacctgcaaagtgcagagcaacagagtgttctgtgacaccatgaacagcctgacactgcccagcgaggtgaacctgtgcaacgttgacatcttcaaccccaaatacgactgcaagatcatgacctctaagaccgacgtgtccagcagcgtgatcaccagcctgggcgccatcgtgtcctgctacggcaagaccaagtgcacagctagcaacaagaaccggggcatcatcaagacattcagcaatggctgcgactacgtgtccaataagggcgtggacaccgtcagcgtcggcaacaccctgtactatgtgaacaagcaggagggaaagagcctgtacgtgaaaggcgagcctatcatcaacttctacgatcctctggtgttccctagctgtgaattctgcgccagcatcagccaggtgaacgagaagatcaaccagagcctggccttcatcagaaagagcgatgagctgctgcacaacgtgaacgccgtgaagagcaccaccaacatcatgattaccaccatcatcatcgtcatcattgtgatcctgctgagcctgatcgccgtgggtcttctgctgtattgcatgaaacagatcgaagataagatcgaggagatcctgagcaagatctaccacatcgagaatgagatcgccagaatcaagaagctcatcggcgagagatga

SEQ ID NO: 92 - RNA, 1743 nt, synthetic construct
  source 1..1743: mol_type = other RNA
atggaactcttaatcctgaaagccaacgctatcaccaccatcctgaccgccgtgaccttctgcttcgccagcggccagaacatcacagaagagttctaccagagcacctgtagcgccgtctccaaaggctacctgagcgctctgagaaccggctggtatacaagcgtgatcaccatcgaactgtccaacatcaagaaaaacaagtgtaacggaacagacgccaagatcaagctgatcaagcaggagctggataagtataagaacgccgtgaccgagctccagctgctgatgcagagcacacctgccaccaacaacagggccagaagagagctgcctcggttcatgaactacacactgaacaatgctaagaaaaccaacgtgacactgagcaagaaaagaaagcggagattcctgggcttcctgctgggcgtgggcagtgccatcgccagcggcgtggccgtgtgcaaagtgctgcacctggaaggcgaggtgaataagatcaaatctgcactgctcagcaccaacaaggccgtggtgtccctgtcgaatggcgtttctgtgctgacttttaaggtgcttgatctgaagaactacatcgacaagcagctgctgcctatcctgaacaagcagagctgttctatcagcaacatcgagacagtgatcgaattccagcaaaaaaacaaccggctgctggaaatcactagagaattcagcgtgaacgctggagtgaccactcccgtgtctacctacatgctgacaaattctgagctgctgagcctgatcaacgacatgcctatcaccaatgaccaaaagaagctgatgtccaacaacgttcaaatcgtgcggcagcagagctacagcatcatgtgcatcatcaaagaggaagtgctggcctacgtggtgcagctgcctctgtacggtgtgatcgacaccccttgctggaagctgcacaccagcccactgtgtaccacaaacaccaaagaaggcagcaatatttgcctgacccggaccgatagaggatggtactgcgataacgctggcagcgtgtcatttttcccccaggccgaaacctgcaaggtgcagtccaaccgcgtgttttgtgataccatgaacagcctgaccctgccatctgaggtgaacctgtgcaatgtggacatcttcaaccccaagtacgactgcaagatcatgaccagcaagaccgacgtcagcagcagcgtgatcacctctctgggcgccattgtgagctgctacggcaagaccaagtgcaccgcctccaataagaatagaggcatcattaagacatttagcaatggctgcgactacgtgtccaacaagggcgtggacaccgtgagcgtgggcaacaccctgtactacgtgaacaagcaggagggcaagtcgctgtacgttaagggagagcctatcatcaacttctacgaccccctggtgttccctagcgacgagttcgacgctagcatctctcaggtgaacgagaagatcaaccagtccctggccttcatcagaaagtctgatgagctgctgcacaacgtcaacgccgtgaagtctacaacaaacatcatgatcacaaccatcatcattgtgatcatcgtgatcctgctgtctctgatcgccgttggcctgctgctgtattgtagcgccatcggcggatacatccccgaggcccctagagatggccaggcttacgtgcggaaggacggcgagtgggtcctgcttagcacattcctg

SEQ ID NO: 93 - RNA, 1743 nt, synthetic construct
  source 1..1743: mol_type = other RNA
atggaactgctgatcctgaaggccaacgctatcaccaccatcctgaccgccgtgacattctgcttcgcctctggccagaacatcacagaggaattctaccagagcacatgttctgccgtgagcaagggctacctgagcgccctgagaaccggctggtacaccagcgtgatcactatcgagctgagcaacatcaagaagaacaagtgcaacggaaccgatgccaagatcaaactgattaagcaggagctggacaagtacaagaacgccgtaaccgagctgcagctgctgatgcagtctacccctgccacaaacaaccgggccagacgggagctgcctagattcatgaactacacactcaacaacgctaagaaaaccaacgtgaccctgtccaagaagcggaaaagacgcttcctgggcttcctgctgggcgtgggcagcgccatcgccagcggcgtcgccgtgtgcaaggtgctgcacctggaaggcgaggtgaataagatcaaaagcgccctgctgtccacaaacaaagctgttgtgtctctgagcaacggagtttccgtcctgaccttcaaagtgctggacctgaaaaattacatcgacaagcaactgctgcctatcctgaacaagcagagctgtagcatcagcaacatcgaaacggtgatcgagtttcagcaaaagaacaatagactgctggaaatcacaagagaattcagcgtgaacgctggcgtgaccacccctgtgagcacctacatgctgactaacagcgagctgttgtccctgatcaatgatatgcctataaccaacgaccagaagaagctgatgagcaacaacgtgcagattgtgcggcagcagagctacagcatcatgtgcatcatcaaggaagaggtgctggcttacgtggtgcagctgcccctgtacggagtaatcgataccccctgctggaagctgcacaccagccctctgtgcacaacgaacaccaaggaaggcagcaacatctgcctgaccaggaccgatagaggctggtattgtgacaacgccggctctgtgagcttcttcccccaggctgagacctgtaaagtgcagtccaaccgggtgttctgcgacacaatgaattctctgacactcccaagcgaggtgaacctgtgtaacgtggatatcttcaaccctaagtatgattgcaagatcatgaccagcaagaccgacgtgtctagctccgttatcacctccctgggcgccatcgtgagttgctacggtaaaacaaagtgtacagccagcaataagaatcggggtattatcaagacctttagcaacggctgcgactacgtgagcaataagggcgtggacaccgtgtctgtcggaaacaccctgtactacgtgaacaagcaggagggcaagagcctgtacgtgaaaggcgagcctatcatcaatttctacgaccccctggtgtttccatctgacgagttcgacgccagcatttctcaggtgaacgagaagatcaaccagagcctggccttcatcagaaagtctgacgagctgctgcacaacgtgaacgccgtgaaaagcaccacaaatatcatgatcaccacaatcatcatcgtgatcatcgtgatcctgctgagcctgatcgccgtgggactgctgctctactgcagcgccatcggcggctacatccccgaggcccctagagatggccaagcatatgttagaaaggacggcgaatgggtgctgctttccacatttctg

SEQ ID NO: 94 - RNA, 1743 nt, synthetic construct
  source 1..1743: mol_type = other RNA
atggaactgctgatcctgaaggccaacgctatcactacaatcctgacagccgtgacattctgcttcgcctctggccagaacatcacagaggaattctaccagtctacatgcagcgccgtgtccaagggatacctgagcgccctccggaccggctggtacaccagcgtgatcaccatcgagctgagcaacatcaagaagaacaagtgcaacggcaccgacgccaagatcaagctgatcaagcaagagctggataagtacaagaacgccgtgaccgagctgcagctgctgatgcagagcaccccagccaccaacaacagagccagacgagaactgcctaggttcatgaactacacactgaacaacgctaagaagaccaacgtgacgctgtccaagaaaagaaagcggagattcctgggcttcctgctgggagtgggctctgctattgccagcggcgtcgccgtgtgcaaggtgctgcacctggaaggcgaggtgaacaaaatcaaaagcgccctgctcagcacaaataaagccgtcgtgtccctgtctaatggcgtgtctgtgctgacatttaaggtgctggacctgaagaactacatcgacaagcagctgcttccaatcctgaacaagcagagctgtagcatcagcaacatcgagaccgtgatcgagtttcagcaaaagaacaatcggctgctggagatcacaagagaattcagcgttaatgccggcgtgaccacccctgtgtctacatacatgctgacaaattccgagctgctgagcctgatcaacgacatgcctatcaccaatgatcagaaaaaactgatgagcaacaacgtgcagatcgttagacagcagagctacagtatcatgtgcatcatcaaagaggaagtcctggcgtacgtggtccaactgcctctgtatggcgtgatcgacaccccctgctggaagctgcacaccagccctctgtgcaccaccaataccaaggaaggcagcaacatctgcctgaccagaaccgatcggggctggtattgcgacaacgctggcagcgtgagcttcttccctcaggctgaaacctgtaaagtgcagagcaatagagtgttttgcgacaccatgaacagcctgaccctgcctagcgaggtgaacctgtgtaatgtggacatcttcaaccccaagtacgactgcaagatcatgaccagcaagacagacgtgtccagctccgtgatcacctctctgggcgccatcgtctcctgctacggcaaaaccaagtgcaccgccagcaacaagaaccggggcatcatcaagacctttagcaacggatgtgattacgtgtcaaacaagggcgtggataccgtgtccgttggaaataccctctactacgtgaacaagcaggaaggcaagagtctgtacgtgaaaggcgagcctatcatcaacttctacgaccccctggtgttccccagcgatgagttcgacgccagcattagccaggtgaacgagaagatcaaccagtctctggccttcatcagaaagagcgacgagttgcttcacaacgttaacgcagtgaagagcacaacaaacatcatgatcaccacaatcatcatcgtgattatcgtgatcctgctgagcctgatcgccgtgggactgctgctgtactgtagcgctattggaggctacatacccgaggcccctagagatggccaggcctatgtgcgcaaggacggcgaatgggtcctgctgtctaccttcctg

SEQ ID NO: 95 - RNA, 1743 nt, synthetic construct
  source 1..1743: mol_type = other RNA
atggaactgctgatccttaaggccaacgctatcaccacaatcctgacagccgtgaccttttgcttcgcctctggccagaacattactgaggaattctaccagtctacatgcagcgccgtgtccaagggctacctgtctgccctgaggacaggatggtataccagcgtgatcaccattgagctgagcaacatcaagaagaacaagtgcaacggcacagacgccaaaatcaaactgatcaagcaggagttagataagtacaagaacgccgtgaccgagctgcagctgctgatgcagtccacccctgctaccaacaacagagccagacgggaactgcctcggttcatgaattacaccctgaacaacgccaagaaaaccaatgtgaccctgagcaagaaaagaaagcggagatttctgggtttcctgctcggcgtgggatccgccatcgctagcggcgttgctgtgtgcaaggtgctgcacctggaaggagaagtgaacaagatcaagagcgccctgctgagcaccaacaaggccgtcgtgtccctgagcaacggcgtttccgtgctgaccttcaaggtgctggacctgaagaattacatcgacaagcagctgctcccaatcctgaacaaacaaagctgttctatcagcaacatcgagacagtcatcgagtttcagcaaaagaacaatagactcctggaaatcacaagagaattttctgtgaatgccggagtgactacacctgtgagcacctacatgctgaccaacagcgagctactgtccctgatcaacgacatgcctatcacaaatgatcagaagaagctgatgagcaacaacgtgcagatcgtgcgccagcagagctacagcatcatgtgcatcatcaaggaagaggtgctggcttacgtggtgcaactgcctctgtacggcgtgatcgacaccccctgctggaagctgcacaccagccctctgtgcaccaccaataccaaagagggatctaacatctgcctgacaagaaccgacagaggctggtactgcgataacgccggcagcgtgagcttcttcccccaggccgagacctgcaaggtgcagagcaatcgggtgttctgtgatacaatgaacagcctgacactgcctagcgaagtgaatctgtgtaacgtggacatcttcaaccccaagtacgactgcaagataatgacctctaagaccgatgtgtctagcagcgttatcacctccctcggagccattgtgtcttgttacggcaaaacaaagtgtaccgccagcaacaaaaacagaggcatcattaagacattcagcaacggctgcgactacgtgagcaacaaaggcgtggacaccgtgtccgtgggcaacaccctgtactacgtgaataagcaggagggcaagagcctgtacgttaagggcgagcctatcatcaacttctatgaccctctggtgttcccaagcgatgagttcgacgccagcatctcccaggtgaacgagaaaattaaccagagcctggccttcatcagaaagtccgacgagctgctgcacaacgtcaacgctgttaagtctacaaccaacatcatgatcacaaccatcatcatcgtaatcatcgtgatcctgctgtctctgatcgccgtgggcctgctgctgtattgcagcgccatcggcggctacatccccgaggcccctagagatggccaggcctacgtgcggaaggacggcgaatgggtgctgctatctaccttcctg

SEQ ID NO: 96 - RNA, 1698 nt, synthetic construct
  source 1..1698: mol_type = other RNA
atggaactgctcatcctgaaggccaacgccattaccacgatcctgaccgccgtgaccttttgcttcgccagcggccagaacatcaccgaggaattctaccagtctacctgtagcgctgtgtctaagggatacctgagcgccctgagaaccggatggtacacctccgtgatcaccattgagctgtctaacatcaagaagaacaagtgcaatggcaccgacgccaagatcaagctgatcaagcaggagctggataagtacaagaatgctgtgacagagctgcagctgctgatgcagtccacacctgccaccaacaatcgggccagaaggggcggcggaagcggcggaggcagcggcggcggcagcttcctgggcttcctgctcggcgtgggaagcgccatcgctagcggagtcgccgtctgcaaggtgctgcacctggaaggcgaggtgaacaagatcaaaagcgccctgctgtccacaaacaaagccgtggtgtctctgtctaacggcgtgtctgttctgacctttaaagtgctggacctgaaaaactacatagacaagcaactgctgcctatcctgaacaagcagagctgttctattagcaacatcgagacagtgatcgagttccagcagaagaacaaccgcctgctggaaatcacccgggaattcagcgtgaacgccggcgttacaacacctgtgtcaacctacatgctgacgaacagcgagctgttatccctgatcaatgacatgcctatcacaaacgaccagaagaagctgatgagcaacaacgtgcaaatcgtgcggcagcaaagctacagcatcatgtgcatcatcaaagaggaagtgctggcctacgtggtccagctgccactgtacggcgtgatcgacaccccttgctggaagctgcacaccagccccctgtgtaccaccaataccaaggaaggcagcaatatctgcctgacacggaccgatagaggctggtattgcgataacgctggcagcgtgtcctttttcccccaggctgagacatgtaaagtgcagtctaacagagtcttctgcgacaccatgaacagcctgaccttgccctccgaagtgaatctgtgcaacgtggacatcttcaatcccaagtacgattgcaagatcatgaccagcaagacagacgtgagcagctctgtgatcacaagcctgggcgccatcgtgtcctgctacggcaagaccaaatgcacagccagcaacaaaaatagaggcatcattaaaacattcagcaatggttgtgattacgtgtccaacaagggcgtggacacagtgtccgtgggcaacaccctgtactacgtgaacaaacaggagggaaagagcctgtatgtgaagggcgaacctatcatcaacttctacgaccccctggtgttcccatcttgtgaattctgcgccagcatcagccaggtgaacgagaagatcaaccagtctctggccttcatcagaaagagcgacgagctgctccacaacgtgaacgcagttaagtctaccaccaacatcatgatcaccaccatcataatcgtgatcatcgtgatcctgctgagcctgatcgccgtgggcctgctgctgtactgcagcgccatcggcggctacatccctgaggcccctagagatggccaggcttatgttagaaaggacggagagtgggtgctgctgagcacatttctg

SEQ ID NO: 97 - RNA, 1698 nt, synthetic construct
  source 1..1698: mol_type = other RNA
atggaactcctgatcctgaaagccaacgccatcaccacaatcctgaccgccgtgacattctgcttcgccagcggccagaacatcacagaggaattctaccagagcacctgcagcgccgtctccaagggttacctgagcgccctgagaacaggctggtacaccagcgtgatcaccatcgagctgtctaacatcaagaagaataaatgtaacggtacagacgccaagatcaagctgatcaaacaggagctggataagtacaagaacgccgtgaccgagctgcagctgctcatgcagagcacccctgccaccaacaacagagccagaaggggaggaggctcaggcggcgggtccggcggaggcagcttcctcggcttcctgctcggcgttggcagcgctatcgcctctggcgtggccgtgtgcaaggtgctgcacctggaaggcgaggtgaacaagatcaagagcgccctgctgagcaccaacaaggccgtggtgagcctgagcaacggcgtgtctgttctgacctttaaggtgctggatctgaagaactacatcgacaagcagctgctgccaatcctgaacaagcagagctgttctatcagcaacatcgagacagtgatcgaatttcagcaaaagaataatagactgctggaaatcacccgggaattctctgtgaacgccggcgtcacaacccctgtgagtacctacatgctgaccaacagcgagctgctgagcctgatcaatgacatgcctatcaccaatgaccagaaaaagctgatgagcaacaacgtgcagatcgtgcggcagcagagctacagcatcatgtgcatcatcaaggaagaagtgctggcctacgtcgtgcaactgcctctgtacggcgtgatcgacacaccttgctggaagctgcacaccagccctctatgcaccaccaacaccaaggaaggctctaatatctgcctgacaagaaccgatagaggctggtattgtgacaacgctggctccgtgtcatttttcccccaggctgaaacctgtaaagtgcagtctaaccgggtgttctgtgataccatgaacagcctgacactgccatctgaggtgaacctgtgtaacgtggacatcttcaaccccaagtacgattgcaagattatgacatctaagaccgacgtgtctagcagcgtgattaccagcctgggcgccatcgtgtcttgctacggcaagacaaagtgcacagccagcaacaaaaatcggggcatcatcaagaccttcagcaatggctgcgactacgtgagcaacaagggagtggacaccgtgagcgtgggcaacaccctgtactacgtgaataaacaggagggaaaatccctgtatgtgaagggcgagcctatcatcaacttctacgaccccctggtcttccctagctgcgagttttgcgccagcatctcccaggtgaacgagaagatcaaccagtccctggctttcatcagaaagagcgacgagctgctgcacaacgtgaacgccgtgaaaagcaccaccaacatcatgatcacaacaattatcatcgtgattatcgtgatcctgctgagcctgatcgccgtcggcctgctgctgtactgcagcgctatcggcggctacatccccgaggcccctagagatggccaagcttacgtgcggaaggacggagagtgggtgctgctgagcacattcctg

SEQ ID NO: 98 - RNA, 1698 nt, synthetic construct
  source 1..1698: mol_type = other RNA
atggaactcctcatcctgaaggccaacgctatcacaaccattctgaccgccgtgacattttgcttcgccagcggccagaacatcacggaggaattctaccagagcacatgttccgcagtgtccaagggctacctgtctgccctgcggacaggctggtacaccagcgtcatcaccatcgagctgtctaatatcaagaaaaacaagtgcaacggcacagacgccaagatcaagctgatcaaacaggagctggataagtacaagaacgctgtgaccgagctgcagctgctgatgcagagcacccctgccaccaacaaccgcgccaggagaggaggcggcagcggcggcggaagcggcggcggcagcttcctgggcttcctgctgggcgttggatctgccatcgcctctggagtggccgtgtgcaaggtgctgcacctggaaggcgaggtgaacaagattaagtctgctctgctcagcaccaataaggccgtcgtgtctctgagcaacggcgtgagcgtcctgaccttcaaggtgctggacctgaaaaattacatcgacaaacagctgctgcctatcctgaacaagcaaagctgcagcatcagcaacatcgagaccgtgatcgagtttcagcaaaagaacaaccggctgctggaaatcacccgggaattcagcgtgaacgccggcgtgaccacccctgtgagtacctacatgctgaccaatagcgagctgctgtctctgatcaatgacatgcctatcaccaacgaccagaagaagctcatgagcaacaacgtgcagatcgtgcggcagcagagctatagcatcatgtgcatcatcaaggaagaggtgctggcttacgtggtgcagctgcccctgtacggcgtgatcgacaccccttgttggaagctgcacactagccccctgtgtaccacaaataccaaagagggaagcaacatatgcctgacaagaacagatagaggctggtattgcgacaacgctggcagcgtgtccttcttcccacaagccgaaacctgcaaggtgcagtctaacagagtgttctgcgatacaatgaacagcctgacactgcctagcgaggtgaacctgtgtaatgtggacatcttcaaccccaagtacgattgcaaaatcatgaccagcaagacagacgtgagctctagcgtgatcacgagcctgggcgccatcgtgagctgctacggcaagaccaagtgcaccgctagcaataagaatagaggcatcatcaaaaccttttcaaacggttgtgactacgtgagcaacaagggcgtggataccgtgagcgtgggcaacaccctgtattacgtgaacaaacaggagggaaagagcctatacgtgaaaggcgagcctattattaacttctacgaccctctggtgtttccatcttgtgaattctgcgcctctatctctcaggtgaatgagaagatcaaccagagtctggccttcatcagaaagagcgacgaactgctgcacaacgtgaatgccgtcaagagcacaaccaacatcatgatcacaacaatcataatcgtgatcattgttatcctgttgagcctgatcgccgtgggcctgctgctgtactgctccgccataggaggatacatccccgaggcccctagagatggccaggcctacgtcagaaaggacggcgaatgggtgctgctgagcacattcctg

SEQ ID NO: 99 - RNA, 1698 nt, synthetic construct
  source 1..1698: mol_type = other RNA
atggaactgctgatcctgaaggctaacgccatcaccacaatcctgacagccgtgaccttctgcttcgccagcggccagaacatcacagaagagttctaccagagcacctgctccgcagtgtctaagggctacctgtctgctctgagaaccggctggtacaccagcgtgattaccatcgagctgagcaacattaagaagaacaaatgcaacggtacagacgccaagatcaagctgatcaagcaggagctggacaaatacaagaacgccgtcacagaactgcagctgctcatgcagtccacacccgccaccaacaaccgcgccagaagaggcggcggcagcggcggaggaagcggaggcggctcttttctgggcttcttgttgggcgtgggatccgccatcgccagcggcgtggccgtgtgcaaggtgctgcacctggaaggcgaggtgaacaagatcaagtccgccctgctgagcaccaacaaagccgtggtgtccctgagcaatggcgtcagcgtcctgacattcaaggtgctcgacctgaaaaactacatcgataaacagctgctgcccatcctgaacaagcagagctgtagcatcagcaatatcgaaaccgtgattgagtttcagcaaaagaacaacagactgcttgagatcactagggaattttctgtgaacgctggagtgacaacccctgtgtccacgtacatgctgacaaattctgagctgctgagcctgatcaacgacatgcctatcacaaatgaccagaaaaagctgatgagcaacaacgtgcagatcgtgcggcagcagagctacagcatcatgtgcataatcaaggaagaagtgctggcctacgtggtgcaactgcctctgtatggcgttattgacaccccttgttggaagctgcacacctccccactgtgcacaaccaacaccaaggaaggcagcaatatctgcctgacccggaccgatagaggatggtattgcgacaacgccggcagcgtgagcttcttcccccaggccgagacttgtaaagtgcagagcaatagagtgttctgcgataccatgaacagcctgaccctgcctagcgaggtgaacctgtgtaatgtggacatcttcaaccccaagtacgattgcaagatcatgaccagcaagacagatgtgagctctagcgtgatcaccagcctgggcgccatcgtaagctgctacggcaagacaaagtgcaccgcctccaacaagaaccggggcatcatcaaaacattcagcaacggatgtgactacgtgagtaacaagggcgtggacaccgtgtccgtgggcaacaccctgtactacgtcaacaaacaggagggaaagagcctgtacgtgaagggagagcctatcatcaacttctacgaccctctggtgtttccatcttgcgagttctgtgcctctatttctcaggtgaacgagaagatcaaccagtctctggccttcatcagaaagagcgacgagctcctgcacaacgtgaatgctgtgaagtctaccaccaacatcatgatcaccaccatcatcatcgtcatcatcgttatcctgctgagcctgatcgccgtgggcctgttactgtactgcagcgccatcggcggctacatccctgaggcccctagagatggccaagcttatgtgcggaaggacggcgaatgggtgctgcttagcacattcctg

SEQ ID NO: 100 - RNA, 1590 nt, synthetic construct
  source 1..1590: mol_type = other RNA
atggaactgctgattctgaaggccaacgctatcaccaccatcctgacagccgtgaccttttgcttcgcctcaggccagaacatcaccgaggaattctaccagagcacctgcagcgccgtcagcaagggatacctgagtgctctgagaacaggctggtacaccagcgtgattaccatcgagctgtccaacatcaagaaaaacaagtgcaatggcaccgacgccaagataaagctgatcaagcaggagctggacaagtacaagaatgccgtgaccgagctgcagctgctgatgggcggcggaagcggcggcggctctggcggaggcagcggcagcgccatcgccagcggagtcgccgtgtgcaaagtgctgcacctggaaggcgaagtgaataaaatcaagtccgccctgctgtccacaaacaaagccgtggtgtctctgagcaacggtgtgtctgtgctgaccttcaaggtgctggacctgaagaactacatcgataagcaactgttgcctatcctgaacaagcagagctgcagcatcagcaacatcgagacagtgatcgagttccagcaaaaaaacaaccggctgctggagatcacacgggaattctctgtgaacgctggagttaccacccctgtgtctacctacatgctgaccaacagcgagctgctgtccctgatcaacgacatgccaatcacaaacgaccagaaaaagctgatgagcaacaatgtgcagatcgtgagacagcagagctacagcatcatgtgcatcatcaaggaagaagtgctggcctatgtcgtgcagctgcctctgtacggcgttatcgatacaccctgctggaaactgcacaccagccctctgtgtaccacaaataccaaggaaggctccaacatctgcctgaccagaaccgatagaggctggtattgtgacaacgccggcagcgtgtccttcttcccccaggccgagacatgcaaggtgcaaagtaacagagtgttctgcgacaccatgaacagccttacactgcccagcgaggtcaacctgtgcaacgtggacatcttcaaccctaagtacgactgcaagatcatgacatctaagacagatgtgtccagcagcgtgatcacctctctgggcgccatcgtgtcttgttacggcaaaaccaagtgcaccgcctctaacaagaatcggggcatcatcaaaacatttagcaacggatgtgactacgtgagcaataagggcgtggacactgtgagcgtcggcaacaccctgtactacgttaacaagcaggagggcaagagcctgtacgtgaagggcgagcctatcatcaacttctacgatcctctcgtgtttccaagctgtgaattttgcgccagcattagccaggtgaacgagaagatcaaccagagcctggctttcattagaaagagcgacgagctgctgatcatcatcgtgatcatcgtgatcctgctgtccctgatcgccgtgggcctgctcctgtactgttctgctatcggaggctatatccccgaggcccctagagatggccaggcctacgtgcggaaggacggcgagtgggtgctgctgagcaccttcctg

SEQ ID NO: 101 - RNA, 1590 nt, synthetic construct
  source 1..1590: mol_type = other RNA
atggaactgctcatcctgaaggccaacgccatcacaaccatcctgaccgccgtgaccttctgcttcgcctctggccagaacatcacagaagaattctaccagagcacctgttctgccgtgagcaagggctacctgagcgccctgagaacaggctggtacaccagcgtgattaccattgaactgagcaacatcaagaagaacaaatgcaacggcaccgacgccaagatcaagctgattaaacaggagctggataagtacaagaacgccgtcacagagctgcagctgctgatgggcggaggatctggaggcggctccggcggcggcagcggatccgccatcgcctccggcgtggccgtgtgtaaagtgctccacctggaaggggaagtgaacaagatcaaatctgcacttctgagcaccaacaaggccgttgtgagcctgtccaatggcgtgtctgtgctgacctttaaggtgctggacctgaagaattacatcgacaagcaactgctgcccatcctgaacaaacagagctgttctataagcaacatcgagacagtgatcgagtttcagcagaaaaacaatcggctgttagagatcaccagagagttcagcgtgaacgccggcgttacaacccctgtttccacctacatgctgacaaacagcgagctgctcagcctgatcaacgacatgcctatcaccaatgaccagaagaaactgatgagcaacaacgtgcagatcgtcagacagcaatcttatagcataatgtgcatcatcaaggaggaggtgctggcttacgtggtgcagctccctctgtacggcgtaatcgacacaccttgttggaagctgcacaccagccccctgtgcactacaaacaccaaagagggctctaacatctgcctgacaagaaccgatagaggctggtactgcgacaacgctggctcagtctccttcttcccacaagctgaaacctgcaaggtgcagtctaatcgcgtgttctgtgatacgatgaacagcctgaccctgccttctgaagtgaatctgtgcaacgtggatatcttcaaccccaagtacgactgcaagatcatgacatccaagacagacgtgagctccagcgtgatcaccagcctgggcgccatcgtgagctgctacggcaagaccaagtgcaccgcctctaacaagaaccggggcatcatcaagaccttcagcaacggctgcgactatgtgagcaataagggcgtggacaccgtgagcgtgggaaataccctgtactacgtgaacaagcaggagggaaagagcctgtacgtgaagggcgagcctatcattaacttctatgaccctctggtgtttccatcctgtgaattctgcgccagcatcagccaggtgaacgagaagatcaaccagagcctggctttcatcagaaagagcgatgagctgctgatcatcatcgtcatcatcgtgatcctgctgagcctgatcgccgtcggcctgctgctgtactgcagcgctatcggaggctacatccccgaggcccctagagatgggcaggcctacgtgcggaaagacggcgagtgggtgctgctgagtaccttcctg

SEQ ID NO: 102 - RNA, 1590 nt, synthetic construct
  source 1..1590: mol_type = other RNA
atggaactgctgatcctgaaggccaacgctatcaccaccatcctaaccgccgttaccttttgcttcgccagcggacagaacatcaccgaggaattctaccagagcacatgcagcgccgtgtcgaaaggctacctgtctgccctgagaacaggctggtacaccagcgtgatcaccatcgagctgtccaacatcaagaaaaacaagtgtaatggcacagacgccaagatcaagctgattaagcaggagttggataagtacaagaacgcagtgacagagctccagctgctgatgggcggcggcagcggcggtggcagcggcggcggaagcggctctgccatcgcgagcggcgtggccgtctgtaaagtgctgcacctggaaggcgaggtgaataagatcaagtccgctctgctgagcacaaacaaggccgtggtgagcctgagcaacggcgtgtccgtgctgacatttaaggtcctggacctgaagaattacatcgacaagcaactgctccccatcctgaacaagcagtcttgtagcatcagcaatatcgaaaccgtgatcgagtttcagcaaaaaaacaaccggctgctggaaatcactcgggaatttagcgtgaacgccggcgtgaccacacctgtgtccacctacatgctgaccaacagtgagctgctgagcctgatcaacgatatgcctatcaccaacgatcagaagaagctgatgagcaacaacgtgcagatcgtgcggcagcagagctacagcatcatgtgcatcattaaagaggaagtgctggcctatgtggtccagctgcctctgtacggagttatcgacacaccctgctggaagctgcacacatctcctctgtgtaccaccaataccaaggaaggcagcaacatctgcctgacaagaaccgataggggatggtattgtgacaacgctggcagcgtgtcattcttcccacaggctgaaacctgcaaggttcaaagcaacagagtgttctgcgatacaatgaacagcctgacactgccatctgaggtgaatctgtgcaacgtggacatcttcaaccctaagtacgactgcaagattatgaccagcaagaccgacgtgtccagctctgtgatcacatctctgggcgccatcgtgagctgttacggcaagaccaagtgcaccgccagcaacaaaaatagaggcatcatcaaaaccttcagcaatggctgcgattacgtgagcaacaaaggcgtcgacactgtgtccgtgggcaacaccctgtactacgtgaacaagcaggagggaaaaagcctgtatgtgaagggcgagcctatcatcaacttctacgaccccctggtgttccctagctgcgagttctgcgcttctatctctcaggtgaacgagaagatcaaccagagccttgccttcatcagaaagagcgacgagctgcttatcatcattgtgatcatcgtgatcctgctgtctctgatcgccgtgggcctgctgctgtactgcagcgccatcggcggatacatccccgaggcccctagagatggccaggcctacgtgagaaaggacggagaatgggtgctgctgagcaccttcctg

SEQ ID NO: 103 - RNA, 1590 nt, synthetic construct; identical to SEQ ID NO: 102
  source 1..1590: mol_type = other RNA